European Patent Specification EP 3 630 143 B1, published June 7, 2023. Title: VIRUS AND METHOD. Applicant: PsiOxus Therapeutics Limited. The sequence listing filed with the application follows.

SEQUENCE LISTING (27 sequences)

SEQ ID NO: 1 - DNA, 34794 bp, Artificial Sequence
  NG-350A genome sequence
tctatctatataatataccttatagatggaatggtgccaatatgtaaatgaggtgattttaaaaagtgtggatcgtgtggtgattggctgtggggttaacggctaaaaggggcggtgcgaccgtgggaaaatgacgttttgtgggggtggagtttttttgcaagttgtcgcgggaaatgtgacgcataaaaaggcttttttctcacggaactacttagttttcccacggtatttaacaggaaatgaggtagttttgaccggatgcaagtgaaaattgttgattttcgcgcgaaaactgaatgaggaagtgtttttctgaataatgtggtatttatggcagggtggagtatttgttcagggccaggtagactttgacccattacgtggaggtttcgattaccgtgttttttacctgaatttccgcgtaccgtgtcaaagtcttctgtttttacgtaggtgtcagctgatcgctagggtatttatacctcagggtttgtgtcaagaggccactcttgagtgccagcgagaagagttttctcctctgcgccggcagtttaataataaaaaaatgagagatttgcgatttctgcctcaggaaataatctctgctgagactggaaatgaaatattggagcttgtggtgcacgccctgatgggagacgatccggagccacctgtgcagctttttgagcctcctacgcttcaggaactgtatgatttagaggtagagggatcggaggattctaatgaggaagctgtaaatggcttttttaccgattctatgcttttagctgctaatgaagggttagaattagatccgcctttggacacttttgatactccaggggtaattgtggaaagcggtacaggtgtaagaaaattacctgatttgagttccgtggactgtgatttgcactgctatgaagacgggtttcctccgagtgatgaggaggaccatgaaaaggagcagtccatgcagactgcagcgggtgagggagtgaaggctgccaatgttggttttcagttggattgcccggagcttcctggacatggctgtaagtcttgtgaatttcacaggaaaaatactggagtaaaggaactgttatgttcgctttgttatatgagaacgcactgccactttatttacagtaagtgtgtttaagttaaaatttaaaggaatatgctgtttttcacatgtatattgagtgtgagttttgtgcttcttattataggtcctgtgtctgatgctgatgaatcaccatctcctgattctactacctcacctcctgagattcaagcacctgttcctgtggacgtgcgcaagcccattcctgtgaagcttaagcctgggaaacgtccagcagtggaaaaacttgaggacttgttacagggtggggacggacctttggacttgagtacacggaaacgtccaagacaataagtgttccatatccgtgtttacttaaggtgacgtcaatatttgtgtgacagtgcaatgtaataaaaatatgttaactgttcactggtttttattgctttttgggcggggactcaggtatataagtagaagcagacctgtgtggttagctcataggagctggctttcatccatggaggtttgggccattttggaagaccttaggaagactaggcaactgttagagaacgcttcggacggagtctccggtttttggagattctggttcgctagtgaattagctagggtagtttttaggataaaacaggactataaacaagaatttgaaaagttgttggtagattgcccaggactttttgaagctcttaatttgggccatcaggttcactttaaagaaaaagttttatcagttttagacttttcaaccccaggtagaactgctgctgctgtggcttttcttacttttatattagataaatggatcccgcagactcatttcagcaggggatacgttttggatttcatagccacagcattgtggagaacatggaaggttcgcaagatgaggacaatcttaggttactggccagtgcagcctttgggtgtagcgggaatcctgaggcatccaccggtcatgccagcggttctggaggaggaacagcaagaggacaacccgagagccggcctggaccctccagtggaggaggcggagtagctgacttgtctcctgaactgcaacgggtgcttactggatctacgtccactggacgggataggggcgttaagagggagagggcatctagtggtactgatgctagatctgagttggctttaagtttaatgagtcgcagacgtcctgaaaccatttggtggcatgaggttcagaaagagggaagggatgaagtttctgtattgcaggagaaatattcactggaacaggtgaaaacatgttggttggagcctgaggatgattgggaggtggccattaaaaattatgccaagatagctttgaggcctgataaacagtataagattactagacggattaatatccggaatgcttgttacatatctggaaatggggctgaggtggtaatagatactcaagacaaggcagttattagatgctgcatgatggatatgtggcctggggtagtcggtatggaagcagtaacttttgtaaatgttaagtttaggggagatggttataatggaatagtgtttatggccaataccaaacttatattgcatggttgtagcttttttggtttcaacaatacctgtgtagatgcctggggacaggttagtgtacggggatgtagtttctatgcgtgttggattgccacagctggcagaaccaagagtcaattgtctctgaagaaatgcatatttcaaagatgtaacctgggcattctgaatgaaggcgaagcaagggtccgccactgcgcttctacagatactggatgttttattttgattaagggaaatgccagcgtaaagcataacatgatttgcggtgcttccgatgagaggccttatcaaatgctcacttgtgctggtgggcattgtaatatgctggctactgtgcatattgtttcccatcaacgcaaaaaatggcctgtttttgatcacaatgtgatgacgaagtgtaccatgcatgcaggtgggcgtagaggaatgtttatgccttaccagtgtaacatgaatcatgtgaaagtgttgttggaaccagatgccttttccagaatgagcctaacaggaatttttgacatgaacatgcaaatctggaagatcctgaggtatgatgatacgagatcgagggtacgcgcatgcgaatgcggaggcaagcatgccaggttccagccggtgtgtgtagatgtgactgaagatctcagaccggatcatttggttattgcccgcactggagcagagttcggatccagtggagaagaaactgactaaggtgagtattgggaaaactttggggtgggattttcagatggacagattgagtaaaaatttgttttttctgtcttgcagctgtcatgagtggaaacgcttcttttaaggggggagtcttcagcccttatctgacagggcgtctcccatcctgggcaggagttcgtcagaatgttatgggatctactgtggatggaagacccgtccaacccgccaattcttcaacgctgacctatgctactttaagttcttcacctttggacgcagctgcagctgccgccgccgcttctgttgccgctaacactgtgcttggaatgggttactatggaagcatcatggctaattccacttcctctaataacccttctaccctgactcaggacaagttacttgtccttttggcccagctggaggctttgacccaacgtctgggtgaactttctcagcaggtggtcgagttgcgagtacaaactgagtctgctgtcggcacggcaaagtctaaataaaaaaatcccagaatcaatgaataaataaacaagcttgttgttgatttaaaatcaagtgtttttatttcatttttcgcgcacggtatgccctagaccaccgatctctatcattgagaactcggtggattttttccaggatcctatagaggtgggattgaatgtttagatacatgggcattaggccgtctttggggtggagatagctccattgaagggattcatgctccggggtagtgttgtaaatcacccagtcataacaaggtcgcagtgcatggtgttgcacaatatcttttagaagtaggctgattgccacagataagcccttggtgtaggtgtttacaaaccggttgagctgggatgggtgcattcggggtgaaattatgtgcattttggattggatttttaagttggcaatattgccgccaagatcccgtcttgggttcatgttatgaaggaccaccaagacggtgtatccggtacatttaggaaatttatcgtgcagcttggatggaaaagcgtggaaaaatttggagacacccttgtgtcctccaagattttccatgcactcatccatgataatagcaatggggccgtgggcagcggcgcgggcaaacacgttccgtgggtctgacacatcatagttatgttcctgagttaaatcatcataagccattttaatgaatttggggcggagagtaccagattggggtatgaatgttccttcgggccccggagcatagttcccctcacagatttgcatttcccaagctttcagttccgagggtggaatcatgtccacctggggggctatgaaaaacaccgtttctggggcgggggtgattaattgtgatgatagcaaatttctgagcaattgagatttgccacatccggtggggccataaatgattccgattacgggttgcaggtggtagtttagggaacggcaactgccgtcttctcgaagcaagggggccacctcgttcatcatttcccttacatgcatattttcccgcaccaaatccattaggaggcgctctcctcctagtgatagaagttcttgtagtgaggaaaagtttttcagcggtttcagaccgtcagccatgggcattttggagagagtttgctgcaaaagttctagtctgttccacagttcagtgatgtgttctatggcatctcgatccagcagacctcctcgtttcgcgggtttggacggctcctggaatagggtatgagacgatgggcgtccagcgctgccagggttcggtccttccagggtctcagtgttcgagtcagggttgtttccgtcacagtgaaggggtgtgcgcctgcttgggcgcttgccagggtgcgcttcagactcatcctgctggtcgaaaacttctgtcgcttggcgccctgtatgtcggccaagtagcagtttaccatgagttcgtagttgagcgcctcggctgcgtggcctttggcgcggagcttacctttggaagttttcttgcataccgggcagtataggcatttcagcgcatacaacttgggcgcaaggaaaacggattctggggagtatgcatctgcgccgcaggaggcgcaaacagtttcacattccaccagccaggttaaatccggttcattggggtcaaaaacaagttttccgccatattttttgatgcgtttcttacctttggtctccatgagttcgtgtcctcgttgagtgacaaacaggctgtccgtgtccccgtagactgattttacaggcctcttctccagtggagtgcctcggtcttcttcgtacaggaactctgaccactctgatacaaaggcgcgcgtccaggccagcacaaaggaggctatgtgggaggggtagcgatcgttgtcaaccagggggtccaccttttccaaagtatgcaaacacatgtcaccctcttcaacatccaggaatgtgattggcttgtaggtgtatttcacgtgacctggggtccccgctgggggggtataaaagggggcggttctttgctcttcctcactgtcttccggatcgctgtccaggaacgtcagctgttggggtaggtattccctctcgaaggcgggcatgacctctgcactcaggttgtcagtttctaagaacgaggaggatttgatattgacagtgccggttgagatgcctttcatgaggttttcgtccatctggtcagaaaacacaatttttttattgtcaagtttggtggcaaatgatccatacagggcgttggataaaagtttggcaatggatcgcatggtttggttcttttccttgtccgcgcgctctttggcggcgatgttgagttggacatactcgcgtgccaggcacttccattcggggaagatagttgttaattcatctggcacgattctcacttgccaccctcgattatgcaaggtaattaaatccacactggtggccacctcgcctcgaaggggttcattggtccaacagagcctacctcctttcctagaacagaaagggggaagtgggtctagcataagttcatcgggagggtctgcatccatggtaaagattcccggaagtaaatccttatcaaaatagctgatgggagtggggtcatctaaggccatttgccattctcgagctgccagtgcgcgctcatatgggttaaggggactgccccatggcatgggatgggtgagtgcagaggcatacatgccacagatgtcatagacgtagatgggatcctcaaagatgcctatgtaggttggatagcatcgcccccctctgatacttgctcgcacatagtcatatagttcatgtgatggcgctagcagccccggacccaagttggtgcgattgggtttttctgttctgtagacgatctggcgaaagatggcgtgagaattggaagagatggtgggtctttgaaaaatgttgaaatgggcatgaggtagacctacagagtctctgacaaagtgggcataagattcttgaagcttggttaccagttcggcggtgacaagtacgtctagggcgcagtagtcaagtgtttcttgaatgatgtcataacctggttggtttttcttttcccacagttcgcggttgagaaggtattcttcgcgatccttccagtactcttctagcggaaacccgtctttgtctgcacggtaagatcctagcatgtagaactgattaactgccttgtaagggcagcagcccttctctacgggtagagagtatgcttgagcagcttttcgtagcgaagcgtgagtaagggcaaaggtgtctctgaccatgactttgaggaattggtatttgaagtcgatgtcgtcacaggctccctgttcccagagttggaagtctacccgtttcttgtaggcggggttgggcaaagcgaaagtaacatcattgaagagaatcttgccggccctgggcatgaaattgcgagtgatgcgaaaaggctgtggtacttccgctcggttattgataacctgggcagctaggacgatctcgtcgaaaccgttgatgttgtgtcctacgatgtataattctatgaaacgcggcgtgcctctgacgtgaggtagcttactgagctcatcaaaggttaggtctgtggggtcagataaggcgtagtgttcgagagcccattcgtgcaggtgaggattcgctttaaggaaggaggaccagaggtccactgccagtgctgtttgtaactggtcccggtactgacgaaaatgccgtccgactgccattttttctggggtgacgcaatagaaggtttgggggtcctgccgccagcgatcccacttgagttttatggcgaggtcataggcgatgttgacgagccgctggtctccagagagtttcatgaccagcatgaaggggattagctgcttgccaaaggaccccatccaggtgtaggtttccacatcgtaggtgagaaagagcctttctgtgcgaggatgagagccaatcgggaagaactggatctcctgccaccagttggaggaatggctgttgatgtgatggaagtagaactccctgcgacgcgccgagcattcatgcttgtgcttgtacagacggccgcagtagtcgcagcgttgcacgggttgtatctcgtgaatgagttgtacctggcttcccttgacgagaaatttcagtgggaagccgaggcctggcgattgtatctcgtgctttactatgttgtctgcatcggcctgttcatcttctgtctcgatggtggtcatgctgacgagccctcgcgggaggcaagtccagacctcggcgcggcaggggcggagctcgaggacgagagcgcgcaggctggagctgtccagggtcctgagacgctgcggactcaggttagtaggcagtgtcaggagattaacttgcatgatcttttggagggcgtgcgggaggttcagatagtacttgatctcaacgggtccgttggtggagatgtcgatggcttgcagggttccgtgtcccttgggcgctaccaccgtgcccttgtttttcattttggacggcggtggctctgttgcttcttgcatgtttagaagcggtgtcgagggcgcgcaccgggcggcaggggcggctcgggacccggcggcatggctggcagtggtacgtcggcgccgcgcgcgggtaggttctggtactgcgccctgagaagactcgcatgcgcgacgacgcggcggttgacatcctggatctgacgcctctgggtgaaagctaccggccccgtgagcttgaacctgaaagagagttcaacagaatcaatctcggtatcgttgacggcggcttgcctaaggatttcttgcacgtcaccagagttgtcctggtaggcgatctccgccatgaactgctcgatctcttcctcttgaagatctccgcggcccgctctctcgacggtggccgcgaggtcgttggagatgcgcccaatgagttgagagaatgcattcatgcccgcctcgttccagacgcggctgtagaccacggcccccacgggatctctcgcgcgcatgaccacctgggcgaggttgagctccacgtggcgggtgaagaccgcatagttgcataggcgctggaaaaggtagttgagtgtggtggcgatgtgctcggtgacgaagaaatacatgatccatcgtctcagcggcatctcgctgacatcgcccagagcttccaagcgctccatggcctcgtagaagtccacggcaaaattaaaaaactgggagtttcgcgcggacacggtcaactcctcttccagaagacggataagttcggcgatggtggtgcgcacctcgcgctcgaaagcccctgggatttcttcctcaatctcttcttcttccactaacatctcttcctcttcaggtggggctgcaggaggagggggaacgcggcgacgccggcggcgcacgggcagacggtcgatgaatctttcaatgacctctccgcggcggcggcgcatggtttcagtgacggcgcggccgttctcgcgcggtcgcagagtaaaaacaccgccgcgcatctccttaaagtggtgactgggaggttctccgtttgggagggagagggcgctgattatacattttattaattggcccgtagggactgcacgcagagatctgatcgtgtcaagatccacgggatctgaaaacctttcgacgaaagcgtctaaccagtcacagtcacaaggtaggctgagtacggcttcttgtgggcgggggtggttatgtgttcggtctgggtcttctgtttcttcttcatctcgggaaggtgagacgatgctgctggtgatgaaattaaagtaggcagttctaagacggcggatggtggcgaggagcaccaggtctttgggtccggcttgctggatacgcaggcgattggccattccccaagcattatcctgacatctagcaagatctttgtagtagtcttgcatgagccgttctacgggcacttcttcctcacccgttctgccatgcatacgtgtgagtccaaatccgcgcattggttgtaccagtgccaagtcagctacgactctttcggcgaggatggcttgctgtacttgggtaagggtggcttgaaagtcatcaaaatccacaaagcggtggtaagctcctgtattaatggtgtaagcacagttggccatgactgaccagttaactgtctggtgaccagggcgcacgagctcggtgtatttaaggcgcgaataggcgcgggtgtcaaagatgtaatcgttgcaggtgcgcaccagatactggtaccctataagaaaatgcggcggtggttggcggtagagaggccatcgttctgtagctggagcgccaggggcgaggtcttccaacataaggcggtgatagccgtagatgtacctggacatccaggtgattcctgcggcggtagtagaagcccgaggaaactcgcgtacgcggttccaaatgttgcgtagcggcatgaagtagttcattgtaggcacggtttgaccagtgaggcgcgcgcagtcattgatgctctatagacacggagaaaatgaaagcgttcagcgactcgactccgtagcctggaggaacgtgaacgggttgggtcgcggtgtaccccggttcgagacttgtactcgagccggccggagccgcggctaacgtggtattggcactcccgtctcgacccagcctacaaaaatccaggatacggaatcgagtcgttttgctggtttccgaatggcagggaagtgagtcctattttttttttttgccgctcagatgcatcccgtgctgcgacagatgcgcccccaacaacagcccccctcgcagcagcagcagcagcaatcacaaaaggctgtccctgcaactactgcaactgccgccgtgagcggtgcgggacagcccgcctatgatctggacttggaagagggcgaaggactggcacgtctaggtgcgccttcacccgagcggcatccgcgagttcaactgaaaaaagattctcgcgaggcgtatgtgccccaacagaacctatttagagacagaagcggcgaggagccggaggagatgcgagcttcccgctttaacgcgggtcgtgagctgcgtcacggtttggaccgaagacgagtgttgcgggacgaggatttcgaagttgatgaaatgacagggatcagtcctgccagggcacacgtggctgcagccaaccttgtatcggcttacgagcagacagtaaaggaagagcgtaacttccaaaagtcttttaataatcatgtgcgaaccctgattgcccgcgaagaagttacccttggtttgatgcatttgtgggatttgatggaagctatcattcagaaccctactagcaaacctctgaccgcccagctgtttctggtggtgcaacacagcagagacaatgaggctttcagagaggcgctgctgaacatcaccgaacccgaggggagatggttgtatgatcttatcaacattctacagagtatcatagtgcaggagcggagcctgggcctggccgagaaggtggctgccatcaattactcggttttgagcttgggaaaatattacgctcgcaaaatctacaagactccatacgttcccatagacaaggaggtgaagatagatgggttctacatgcgcatgacgctcaaggtcttgaccctgagcgatgatcttggggtgtatcgcaatgacagaatgcatcgcgcggttagcgccagcaggaggcgcgagttaagcgacagggaactgatgcacagtttgcaaagagctctgactggagctggaaccgagggtgagaattacttcgacatgggagctgacttgcagtggcagcctagtcgcagggctctgagcgccgcgacggcaggatgtgagcttccttacatagaagaggcggatgaaggcgaggaggaagagggcgagtacttggaagactgatggcacaacccgtgttttttgctagatggaacagcaagcaccggatcccgcaatgcgggcggcgctgcagagccagccgtccggcattaactcctcggacgattggacccaggccatgcaacgtatcatggcgttgacgactcgcaaccccgaagcctttagacagcaaccccaggccaaccgtctatcggccatcatggaagctgtagtgccttcccgctctaatcccactcatgagaaggtcctggccatcgtgaacgcgttggtggagaacaaagctattcgtccagatgaggccggactggtatacaacgctctcttagaacgcgtggctcgctacaacagtagcaatgtgcaaaccaatttggaccgtatgataacagatgtacgcgaagccgtgtctcagcgcgaaaggttccagcgtgatgccaacctgggttcgctggtggcgttaaatgctttcttgagtactcagcctgctaatgtgccgcgtggtcaacaggattatactaactttttaagtgctttgagactgatggtatcagaagtacctcagagcgaagtgtatcagtccggtcctgattacttctttcagactagcagacagggcttgcagacggtaaatctgagccaagcttttaaaaaccttaaaggtttgtggggagtgcatgccccggtaggagaaagagcaaccgtgtctagcttgttaactccgaactcccgcctattattactgttggtagctcctttcaccgacagcggtagcatcgaccgtaattcctatttgggttacctactaaacctgtatcgcgaagccatagggcaaagtcaggtggacgagcagacctatcaagaaattacccaagtcagtcgcgctttgggacaggaagacactggcagtttggaagccactctgaacttcttgcttaccaatcggtctcaaaagatccctcctcaatatgctcttactgcggaggaggagaggatccttagatatgtgcagcagagcgtgggattgtttctgatgcaagagggggcaactccgactgcagcactggacatgacagcgcgaaatatggagcccagcatgtatgccagtaaccgacctttcattaacaaactgctggactacttgcacagagctgccgctatgaactctgattatttcaccaatgccatcttaaacccgcactggctgcccccacctggtttctacacgggcgaatatgacatgcccgaccctaatgacggatttctgtgggacgacgtggacagcgatgttttttcacctctttctgatcatcgcacgtggaaaaaggaaggcggcgatagaatgcattcttctgcatcgctgtccggggtcatgggtgctaccgcggctgagcccgagtctgcaagtccttttcctagtctacccttttctctacacagtgtacgtagcagcgaagtgggtagaataagtcgcccgagtttaatgggcgaagaggagtatctaaacgattccttgctcagaccggcaagagaaaaaaatttcccaaacaatggaatagaaagtttggtggataaaatgagtagatggaagacttatgctcaggatcacagagacgagcctgggatcatggggattacaagtagagcgagccgtagacgccagcgccatgacagacagaggggtcttgtgtgggacgatgaggattcggccgatgatagcagcgtgctggacttgggtgggagaggaaggggcaacccgtttgctcatttgcgccctcgcttgggtggtatgttgtaaaaaaaaataaaaaaaaaactcaccaaggccatggcgacgagcgtacgttcgttcttctttattatctgtgtctagtataatgaggcgagtcgtgctaggcggagcggtggtgtatccggagggtcctcctccttcgtacgagagcgtgatgcagcagcagcaggcgacggcggtgatgcaatccccactggaggctccctttgtgcctccgcgatacctggcacctacggagggcagaaacagcattcgttattcggaactggcacctcagtacgataccaccaggttgtatctggtggacaacaagtcggcggacattgcttctctgaactatcagaatgaccacagcaacttcttgaccacggtggtgcaaaacaatgactttacccctacggaagccagcacccagaccattaactttgatgaacgatcgcggtggggcggtcagctaaagaccatcatgcatactaacatgccaaacgtgaacgagtatatgtttagtaacaagttcaaagcgcgtgtgatggtgtccagaaaacctcccgacggtgctgcagttggggatacttatgatcacaagcaggatattttgaaatatgagtggttcgagtttactttgccagaaggcaacttttcagttactatgactattgatttgatgaacaatgccatcatagataattacttgaaagtgggtagacagaatggagtgcttgaaagtgacattggtgttaagttcgacaccaggaacttcaagctgggatgggatcccgaaaccaagttgatcatgcctggagtgtatacgtatgaagccttccatcctgacattgtcttactgcctggctgcggagtggattttaccgagagtcgtttgagcaaccttcttggtatcagaaaaaaacagccatttcaagagggttttaagattttgtatgaagatttagaaggtggtaatattccggccctcttggatgtagatgcctatgagaacagtaagaaagaacaaaaagccaaaatagaagctgctacagctgctgcagaagctaaggcaaacatagttgccagcgactctacaagggttgctaacgctggagaggtcagaggagacaattttgcgccaacacctgttccgactgcagaatcattattggccgatgtgtctgaaggaacggacgtgaaactcactattcaacctgtagaaaaagatagtaagaatagaagctataatgtgttggaagacaaaatcaacacagcctatcgcagttggtatctttcgtacaattatggcgatcccgaaaaaggagtgcgttcctggacattgctcaccacctcagatgtcacctgcggagcagagcaggtctactggtcgcttccagacatgatgaaggatcctgtcactttccgctccactagacaagtcagtaactaccctgtggtgggtgcagagcttatgcccgtcttctcaaagagcttctacaacgaacaagctgtgtactcccagcagctccgccagtccacctcgcttacgcacgtcttcaaccgctttcctgagaaccagattttaatccgtccgccggcgcccaccattaccaccgtcagtgaaaacgttcctgctctcacagatcacgggaccctgccgttgcgcagcagtatccggggagtccaacgtgtgaccgttactgacgccagacgccgcacctgtccctacgtgtacaaggcactgggcatagtcgcaccgcgcgtcctttcaagccgcactttctaaaaaaaaaaaaaatgtccattcttatctcgcccagtaataacaccggttggggtctgcgcgctccaagcaagatgtacggaggcgcacgcaaacgttctacccaacatcctgtccgtgttcgcggacattttcgcgctccatggggcgccctcaagggccgcactcgcgttcgaaccaccgtcgatgatgtaatcgatcaggtggttgccgacgcccgtaattatactcctactgcgcctacatctactgtggatgcagttattgacagtgtagtggctgacgctcgcaactatgctcgacgtaagagccggcgaaggcgcattgccagacgccaccgagctaccactgccatgcgagccgcaagagctctgctacgaagagctagacgcgtggggcgaagagccatgcttagggcggccagacgtgcagcttcgggcgccagcgccggcaggtcccgcaggcaagcagccgctgtcgcagcggcgactattgccgacatggcccaatcgcgaagaggcaatgtatactgggtgcgtgacgctgccaccggtcaacgtgtacccgtgcgcacccgtccccctcgcacttagaagatactgagcagtctccgatgttgtgtcccagcggcgaggatgtccaagcgcaaatacaaggaagaaatgctgcaggttatcgcacctgaagtctacggccaaccgttgaaggatgaaaaaaaaccccgcaaaatcaagcgggttaaaaaggacaaaaaagaagaggaagatggcgatgatgggctggcggagtttgtgcgcgagtttgccccacggcgacgcgtgcaatggcgtgggcgcaaagttcgacatgtgttgagacctggaacttcggtggtctttacacccggcgagcgttcaagcgctacttttaagcgttcctatgatgaggtgtacggggatgatgatattcttgagcaggcggctgaccgattaggcgagtttgcttatggcaagcgtagtagaataacttccaaggatgagacagtgtcgatacccttggatcatggaaatcccacccctagtcttaaaccggtcactttgcagcaagtgttacccgtaactccgcgaacaggtgttaaacgcgaaggtgaagatttgtatcccactatgcaactgatggtacccaaacgccagaagttggaggacgttttggagaaagtaaaagtggatccagatattcaacctgaggttaaagtgagacccattaagcaggtagcgcctggtctgggggtacaaactgtagacattaagattcccactgaaagtatggaagtgcaaactgaacccgcaaagcctactgccacctccactgaagtgcaaacggatccatggatgcccatgcctattacaactgacgccgccggtcccactcgaagatcccgacgaaagtacggtccagcaagtctgttgatgcccaattatgttgtacacccatctattattcctactcctggttaccgaggcactcgctactatcgcagccgaaacagtacctcccgccgtcgccgcaagacacctgcaaatcgcagtcgtcgccgtagacgcacaagcaaaccgactcccggcgccctggtgcggcaagtgtaccgcaatggtagtgcggaacctttgacactgccgcgtgcgcgttaccatccgagtatcatcacttaatcaatgttgccgctgcctccttgcagatatggccctcacttgtcgccttcgcgttcccatcactggttaccgaggaagaaactcgcgccgtagaagagggatgttgggacgcggaatgcgacgctacaggcgacggcgtgctatccgcaagcaattgcggggtggttttttaccagccttaattccaattatcgctgctgcaattggcgcgataccaggcatagcttccgtggcggttcaggcctcgcaacgacattgacattggaaaaaaacgtataaataaaaaaaaaaaaatacaatggactctgacactcctggtcctgtgactatgttttcttagagatggaagacatcaatttttcatccttggctccgcgacacggcacgaagccgtacatgggcacctggagcgacatcggcacgagccaactgaacgggggcgccttcaattggagcagtatctggagcgggcttaaaaattttggctcaaccataaaaacatacgggaacaaagcttggaacagcagtacaggacaggcgcttagaaataaacttaaagaccagaacttccaacaaaaagtagtcgatgggatagcttccggcatcaatggagtggtagatttggctaaccaggctgtgcagaaaaagataaacagtcgtttggacccgccgccagcaaccccaggtgaaatgcaagtggaggaagaaattcctccgccagaaaaacgaggcgacaagcgtccgcgtcccgatttggaagagacgctggtgacgcgcgtagatgaaccgccttcttatgaggaagcaacgaagcttggaatgcccaccactagaccgatagccccaatggccaccggggtgatgaaaccttctcagttgcatcgacccgtcaccttggatttgccccctccccctgctgctactgctgtacccgcttctaagcctgtcgctgccccgaaaccagtcgccgtagccaggtcacgtcccgggggcgctcctcgtccaaatgcgcactggcaaaatactctgaacagcatcgtgggtctaggcgtgcaaagtgtaaaacgccgtcgctgcttttaattaaatatggagtagcgcttaacttgcctatctgtgtatatgtgtcattacacgccgtcacagcagcagaggaaaaaaggaagaggtcgtgcgtcgacgctgagttactttcaagatggccaccccatcgatgctgccccaatgggcatacatgcacatcgccggacaggatgcttcggagtacctgagtccgggtctggtgcagttcgcccgcgccacagacacctacttcaatctgggaaataagtttagaaatcccaccgtagcgccgacccacgatgtgaccaccgaccgtagccagcggctcatgttgcgcttcgtgcccgttgaccgggaggacaatacatactcttacaaagtgcggtacaccctggccgtgggcgacaacagagtgctggatatggccagcacgttctttgacattaggggtgtgttggacagaggtcccagtttcaaaccctattctggtacggcttacaactccctggctcctaaaggcgctccaaatacatctcagtggattgcagaaggtgtaaaaaatacaactggtgaggaacacgtaacagaagaggaaaccaatactactacttacacttttggcaatgctcctgtaaaagctgaagctgaaattacaaaagaaggactcccagtaggtttggaagtttcagatgaagaaagtaaaccgatttatgctgataaaacatatcagccagaacctcagctgggagatgaaacttggactgaccttgatggaaaaaccgaaaagtatggaggcagggctctcaaacccgatactaagatgaaaccatgctacgggtcctttgccaaacctactaatgtgaaaggcggtcaggcaaaacaaaaaacaacggagcagccaaatcagaaagtcgaatatgatatcgacatggagttttttgatgcggcatcgcagaaaacaaacttaagtcctaaaattgtcatgtatgcagaaaatgtaaatttggaaactccagacactcatgtagtgtacaaacctggaacagaagacacaagttccgaagctaatttgggacaacaatctatgcccaacagacccaactacattggcttcagagataactttattggacttatgtactataacagtactggtaacatgggggtgctggctggtcaagcgtctcagttaaatgcagtggttgacttgcaggacagaaacacagaactttcttaccaactcttgcttgactctctgggcgacagaaccagatactttagcatgtggaatcaggctgtggacagttatgatcctgatgtacgtgttattgaaaatcatggtgtggaagatgaacttcccaactactgttttccactggacggcataggtgttccaacaaccagttacaaatcaatagttccaaatggagacaatgcgcctaattggaaggaacctgaagtaaatggaacaagtgagatcggacagggtaatttgtttgccatggaaattaaccttcaagccaatctatggcgaagtttcctttattccaatgtggctctatatctcccagactcgtacaaatacaccccgtccaatgtcactcttccagaaaacaaaaacacctacgactacatgaacgggcgggtggtgccgccatctctagtagacacctatgtgaacattggtgccaggtggtctctggatgccatggacaatgtcaacccattcaaccaccaccgtaacgctggcttgcgttaccgatccatgcttctgggtaacggacgttatgtgcctttccacatacaagtgcctcaaaaattcttcgctgttaaaaacctgctgcttctcccaggctcctacacttatgagtggaactttaggaaggatgtgaacatggttctacagagttccctcggtaacgacctgcgggtagatggcgccagcatcagtttcacgagcatcaacctctatgctacttttttccccatggctcacaacaccgcttccacccttgaagccatgctgcggaatgacaccaatgatcagtcattcaacgactacctatctgcagctaacatgctctaccccattcctgccaatgcaaccaatattcccatttccattccttctcgcaactgggcggctttcagaggctggtcatttaccagactgaaaaccaaagaaactccctctttggggtctggatttgacccctactttgtctattctggttctattccctacctggatggtaccttctacctgaaccacacttttaagaaggtttccatcatgtttgactcttcagtgagctggcctggaaatgacaggttactatctcctaacgaatttgaaataaagcgcactgtggatggcgaaggctacaacgtagcccaatgcaacatgaccaaagactggttcttggtacagatgctcgccaactacaacatcggctatcagggcttctacattccagaaggatacaaagatcgcatgtattcatttttcagaaacttccagcccatgagcaggcaggtggttgatgaggtcaattacaaagacttcaaggccgtcgccataccctaccaacacaacaactctggctttgtgggttacatggctccgaccatgcgccaaggtcaaccctatcccgctaactatccctatccactcattggaacaactgccgtaaatagtgttacgcagaaaaagttcttgtgtgacagaaccatgtggcgcataccgttctcgagcaacttcatgtctatgggggcccttacagacttgggacagaatatgctctatgccaactcagctcatgctctggacatgacctttgaggtggatcccatggatgagcccaccctgctttatcttctcttcgaagttttcgacgtggtcagagtgcatcagccacaccgcggcatcatcgaggcagtctacctgcgtacaccgttctcggccggtaacgctaccacgtaagaagcttcttgcttcttgcaaatagcagctgcaaccatggcctgcggatcccaaaacggctccagcgagcaagagctcagagccattgtccaagacctgggttgcggaccctattttttgggaacctacgataagcgcttcccggggttcatggcccccgataagctcgcctgtgccattgtaaatacggccggacgtgagacggggggagagcactggttggctttcggttggaacccacgttctaacacctgctacctttttgatccttttggattctcggatgatcgtctcaaacagatttaccagtttgaatatgagggtctcctgcgccgcagcgctcttgctaccaaggaccgctgtattacgctggaaaaatctacccagaccgtgcagggtccccgttctgccgcctgcggacttttctgctgcatgttccttcacgcctttgtgcactggcctgaccgtcccatggacggaaaccccaccatgaaattgctaactggagtgccaaacaacatgcttcattctcctaaagtccagcccaccctgtgtgacaatcaaaaagcactctaccattttcttaatacccattcgccttattttcgctcccatcgtacacacatcgaaagggccactgcgttcgaccgtatggatgttcaataatgactcatgtaaacaacgtgttcaataaacatcactttatttttttacatgtatcaaggctctgcattacttatttatttacaagtcgaatgggttctgacgagaatcagaatgacccgcaggcagtgatacgttgcggaactgatacttgggttgccacttgaattcgggaatcaccaacttgggaaccggtatatcgggcaggatgtcactccacagctttctggtcagctgcaaagctccaagcaggtcaggagccgaaatcttgaaatcacaattaggaccagtgctttgagcgcgagagttgcggtacaccggattgcagcactgaaacaccatcagcgacggatgtctcacgcttgccagcacggtgggatctgcaatcatgcccacatccagatcttcagcattggcaatgctgaacggggtcatcttgcaggtctgcctacccatggcgggcacccaattaggcttgtggttgcaatcgcagtgcagggggatcagtatcatcttggcctgatcctgtctgattcctggatacacggctctcatgaaagcatcatattgcttgaaagcctgctgggctttactaccctcggtataaaacatcccgcaggacctgctcgaaaactggttagctgcacagccggcatcattcacacagcagcgggcgtcattgttagctatttgcaccacacttctgccccagcggttttgggtgattttggttcgctcgggattctcctttaaggctcgttgtccgttctcgctggccacatccatctcgataatctgctccttctgaatcataatattgccatgcaggcacttcagcttgccctcataatcattgcagccatgaggccacaacgcacagcctgtacattcccaattatggtgggcgatctgagaaaaagaatgtatcattccctgcagaaatcttcccatcatcgtgctcagtgtcttgtgactagtgaaagttaactggatgcctcggtgctcctcgtttacgtactggtgacagatgcgcttgtattgttcgtgttgctcaggcattagtttaaaagaggttctaagttcgttatccagcctgtacttctccatcagcagacacatcacttccatgcctttctcccaagcagacaccaggggcaagctaatcggattcttaacagtgcaggcagcagctcctttagccagagggtcatctttagcgatcttctcaatgcttcttttgccatccttctcaacgatgcgcacgggcgggtagctgaaacccactgctacaagttgcgcctcttctctttcttcttcgctgtcttgactgatgtcttgcatggggatatgtttggtcttccttggcttctttttggggggtatcggaggaggaggactgtcgctccgttccggagacagggaggattgtgacgtttcgctcaccattaccaactgactgtcggtagaagaacctgaccccacacggcgacaggtgtttctcttcgggggcagaggtggaggcgattgcgaagggctgcggtccgacctggaaggcggatgactggcagaaccccttccgcgttcgggggtgtgctccctgtggcggtcgcttaactgatttccttcgcggctggccattgtgttctcctaggcagagaaacaacagacatggaaactcagccattgctgtcaacatcgccacgagtgccatcacatctcgtcctcagcgacgaggaaaaggagcagagcttaagcattccaccgcccagtcctgccaccacctctaccctagaagataaggaggtcgacgcatctcatgacatgcagaataaaaaagcgaaagagtctgagacagacatcgagcaagacccgggctatgtgacaccggtggaacacgaggaagagttgaaacgctttctagagagagaggatgaaaactgcccaaaacaacgagcagataactatcaccaagatgctggaaatagggatcagaacaccgactacctcatagggcttgacggggaagacgcgctccttaaacatctagcaagacagtcgctcatagtcaaggatgcattattggacagaactgaagtgcccatcagtgtggaagagctcagccgcgcctacgagcttaacctcttttcacctcgtactccccccaaacgtcagccaaacggcacctgcgagccaaatcctcgcttaaacttttatccagcttttgctgtgccagaagtactggctacctatcacatcttttttaaaaatcaaaaaattccagtctcctgccgcgctaatcgcacccgcgccgatgccctactcaatctgggacctggttcacgcttacctgatatagcttccttggaagaggttccaaagatcttcgagggtctgggcaataatgagactcgggccgcaaatgctctgcaaaagggagaaaatggcatggatgagcatcacagcgttctggtggaattggaaggcgataatgccagactcgcagtactcaagcgaagcatcgaggtcacacacttcgcatatcccgctgtcaacctgccccctaaagtcatgacggcggtcatggaccagttactcattaagcgcgcaagtcccctttcagaagacatgcatgacccagatgcctgtgatgagggtaaaccagtggtcagtgatgagcagctaacccgatggctgggcaccgactctcccagggatttggaagagcgtcgcaagcttatgatggccgtggtgctggttaccgtagaactagagtgtctccgacgtttctttaccgattcagaaaccttgcgcaaactcgaagagaatctgcactacacttttagacacggctttgtgcggcaggcatgcaagatatctaacgtggaactcaccaacctggtttcctacatgggtattctgcatgagaatcgcctaggacaaagcgtgctgcacagcaccctgaagggggaagcccgccgtgattacatccgcgattgtgtctatctgtacctgtgccacacgtggcaaaccggcatgggtgtatggcagcaatgtttagaagaacagaacttgaaagagcttgacaagctcttacagaaatctcttaaggttctgtggacagggttcgacgagcgcaccgtcgcttccgacctggcagacctcatcttcccagagcgtctcagggttactttgcgaaacggattgcctgactttatgagccagagcatgcttaacaattttcgctctttcatcctggaacgctccggtatcctgcccgccacctgctgcgcactgccctccgactttgtgcctctcacctaccgcgagtgccccccgccgctatggagtcactgctacctgttccgtctggccaactatctctcctaccactcggatgtgatcgaggatgtgagcggagacggcttgctggagtgtcactgccgctgcaatctgtgcacgccccaccggtccctagcttgcaacccccagttgatgagcgaaacccagataataggcacctttgaattgcaaggccccagcagccaaggcgatgggtcttctcctgggcaaagtttaaaactgaccccgggactgtggacctccgcctacttgcgcaagtttgctccggaagattaccacccctatgaaatcaagttctatgaggaccaatcacagcctccaaaggccgaactttcggcctgcgtcatcacccagggggcaattctggcccaattgcaagccatccaaaaatcccgccaagaatttctactgaaaaagggtaagggggtctaccttgacccccagaccggcgaggaactcaacacaaggttccctcaggatgtcccaacgacgagaaaacaagaagttgaaggtgcagccgccgcccccagaagatatggaggaagattgggacagtcaggcagaggaggcggaggaggacagtctggaggacagtctggaggaagacagtttggaggaggaaaacgaggaggcagaggaggtggaagaagtaaccgccgacaaacagttatcctcggctgcggagacaagcaacagcgctaccatctccgctccgagtcgaggaacccggcggcgtcccagcagtagatgggacgagaccggacgcttcccgaacccaaccagcgcttccaagaccggtaagaaggatcggcagggatacaagtcctggcgggggcataagaatgccatcatctcctgcttgcatgagtgcgggggcaacatatccttcacgcggcgctacttgctattccaccatggggtgaactttccgcgcaatgttttgcattactaccgtcacctccacagcccctactatagccagcaaatcccggcagtctcgacagataaagacagcggcggcgacctccaacagaaaaccagcagcggcagttagaaaatacacaacaagtgcagcaacaggaggattaaagattacagccaacgagccagcgcaaacccgagagttaagaaatcggatctttccaaccctgtatgccatcttccagcagagtcggggtcaagagcaggaactgaaaataaaaaaccgatctctgcgttcgctcaccagaagttgtttgtatcacaagagcgaagatcaacttcagcgcactctcgaggacgccgaggctctcttcaacaagtactgcgcgctgactcttaaagagtaggcagcgaccgcgcttattcaaaaaaggcgggaattacatcatcctcgacatgagtaaagaaattcccacgccttacatgtggagttatcaaccccaaatgggattggcggcaggcgcctcccaggactactccacccgcatgaattggctcagcgccgggccttctatgatttctcgagttaatgatatacgcgcctaccgaaaccaaatacttttggaacagtcagctcttaccaccacgccccgccaacaccttaatcccagaaattggcccgccgccctagtgtaccaggaaagtcccgctcccaccactgtattacttcctcgagacgcccaggccgaagtccaaatgactaatgcaggtgcgcagttagctggcggctccaccctatgtcgtcacaggcctcggcataatataaaacgcctgatgatcagaggccgaggtatccagctcaacgacgagtcggtgagctctccgcttggtctacgaccagacggaatctttcagattgccggctgcgggagatcttccttcacccctcgtcaggctgttctgactttggaaagttcgtcttcgcaaccccgctcgggcggaatcgggaccgttcaatttgtggaggagtttactccctctgtctacttcaaccccttctccggatctcctgggcattacccggacgagttcataccgaacttcgacgcgattagcgagtcagtggacggctacgattgatgtctggtgacgcggctgagctatctcggctgcgacatctagaccactgccgccgctttcgctgctttgcccgggaactcattgagttcatctacttcgaactccccaaggatcaccctcaaggtccggcccacggagtgcggatttctatcgaaggcaaaatagactctcgcctgcaacgaattttctcccagcggcccgtgctgatcgagcgagaccagggaaacaccacggtttccatctactgcatttgtaatcaccccggattgcatgaaagcctttgctgtcttatgtgtactgagtttaataaaaactgaattaagactctcctacggactgccgcttcttcaacccggattttacaaccagaagaacgaaacttttcctgtcgtccaggactctgttaacttcacctttcctactcacaaactagaagctcaacgactacaccgcttttccagaagcattttccctactaatactactttcaaaaccggaggtgagctccaaggtcttcctacagaaaacccttgggtggaagcgggccttgtagtgctaggaattcttgcgggtgggcttgtgattattctttgctacctatacacaccttgcttcactttcttagtggtgttgtggtattggtttaaaaaatggggcccatactagtcttgcttgttttactttcgcttttggaaccgggttctgccaattacgatccatgtctagacttcgacccagaaaactgcacacttacttttgcacccgacacaagccgcatctgtggagttcatcgcctctcttacgaacttggcccccaacgacaaaaatttacctgcatggtgggaatcaaccccatagttatcacccagcaaagtggagatactaagggttgcattcactgctcctgcgattccatcgagtgcacctacaccctgctgaagaccctatgcggcctaagagacctgctaccaatgaattaaaaaatgattaataaaaaatcacttacttgaaatcagcaataaggtctctgttgaaattttctcccagcagcacctcacttccctcttcccaactctggtattctaaaccccgttcagcggcatactttctccatactttaaaggggatgtcaaattttagctcctctcctgtacccacaatcttcatgtctttcttcccagatgaccaagagagtccggctcagtgactccttcaaccctgtctacccctatgaagatgaaagcacctcccaacacccctttataaacccagggtttatttccccaaatggcttcacacaaagcccaaacggagttcttactttaaaatgtttaaccccactaacaaccacaggcggatctctacagctaaaagtgggagggggacttacagtggatgacaccaacggttttttgaaagaaaacataagtgccaccacaccactcgttaagactggtcactctataggtttaccactaggagccggattgggaacgaatgaaaataaactttgtatcaaattaggacaaggacttacattcaattcaaacaacatttgcattgatgacaatattaacaccttatggacaggagtcaaccccaccgaagccaactgtcaaatcatgaactccagtgaatctaatgattgcaaattaattctaacactagttaaaactggagcactagtcactgcatttgtttatgttataggagtatctaacaattttaatatgctaactacacacagaaatataaattttactgcagagctgtttttcgattctactggtaatttactaactagactctcatccctcaaaactccacttaatcataaatcaggacaaaacatggctactggtgccattactaatgctaaaggtttcatgcccagcacgactgcctatcctttcaatgataattctagagaaaaagaaaactacatttacggaacttgttactacacagctagtgatcgcactgcttttcccattgacatatctgtcatgcttaaccgaagagcaataaatgacgagacatcatattgtattcgtataacttggtcctggaacacaggagatgccccagaggtgcaaacctctgctacaaccctagtcacctccccatttaccttttactacatcagagaagacgactgacaaataaagtttgcgatcgccaggcccaccatggactggacctggcgcatcctgttcttggtggcagctgctacgggagctcattcccaggtgcagctggtgcaatccggcgctgaggtgaagaaacccggggcttcagtcaaagtcagctgcaaggctagcggctacacctttactggctattacatgcactgggtgaggcaggctccgggacagggtctggaatggatgggatggatcaatccggacagcggcgggaccaattacgcacaaaagttccaaggccgcgtgacgatgacccgggacacttcgatctcaaccgcctacatggagctgaaccgcctgaggtcggatgacaccgctgtgtactactgcgctcgcgaccaacccctggggtactgcaccaacggagtgtgttcatacttcgactactggggccaaggcacgctggtcactgtgtcatcggcgtccactaagggcccgtcggtcttcccactagctccgtgctcgcggtcgacttcggaatcaactgcggcactcggatgccttgtcaaggactacttcccagaacccgtgaccgtctcgtggaactcaggcgccctgacgagcggtgtccacactttcccggcggtgctgcagtcatcggggctatacagcctgagcagcgtggttactgtgccgtcatcaaacttcgggacccagacttacacttgcaatgtggaccacaagccgtcaaataccaaagtggacaagactgtggaacgcaaatgttgcgtggaatgccctccgtgcccggcccccccagtcgctggcccatccgtgttcctcttccctccgaagccaaaagacactctgatgatttcgagaactccggaggtcacttgcgtggtggtcgacgtgtcgcacgaggatccagaggtgcagttcaactggtacgtggatggagtggaggtgcacaatgccaagaccaagccgcgcgaagaacaattcaactccacctttcgggtcgtgtccgtgctgaccgtggtacaccaagactggctgaacggaaaggagtacaaatgcaaggtgagcaacaaggggctgccggctccaatcgaaaagaccatctcaaagactaaggggcaacctcgcgagccacaggtgtataccctgcctccaagcagggaggaaatgaccaaaaaccaggtgagcctgacctgtctggtgaagggcttttaccccagcgacatcgccgtcgagtgggaaagcaacggacaacccgagaacaactacaagaccactccgcccatgctggactccgacgggtcatttttcctgtactcaaagctgactgtggacaagtcccggtggcagcaaggtaacgtgttctcctgctcggtgatgcacgaagctttgcacaaccactacactcaaaagtcactttccttgtcaccgggcaaggggtcgggcgccactaacttttccttgctcaagcaggcgggcgatgtggaggagaatccgggcccgcgcctcccggcgcaactgctgggcctcctcctcctctggtttcccggctcccgctgtgacatccagatgactcagtcgcccagctccgtgtccgcatcggtgggggacagagtcaccatcacctgcagagcttcacaagggatctattcctggctggcgtggtatcagcagaagcctggaaaggcccccaacctcctgatttacaccgcatcgactctccagtcaggcgtgccatcccggttctcagggtccggctccggaaccgacttcactctgactatcagctccctgcaaccagaagatttcgctacctactactgccagcaggcaaacatctttccgctaactttcggcggaggcacgaaggtggagatcaagagaaccgtggcggccccttccgtcttcatcttcccaccgtcagacgaacaactcaaatccggtaccgcctccgtcgtgtgcctgctcaataacttctatccacgcgaggccaaggtccagtggaaagtggataacgccctgcagtccggaaacagccaggagtcagtgaccgaacaggattccaaggacagcacttactcgctctcaagcaccctcaccctgtcgaaggcggattacgagaagcacaaagtctacgcctgcgaagtgactcatcaaggactctcatcaccggtaactaagagcttcaatcgcggagaatgctaggctagcttgactgactgagatacagcgtaccttcagctcacagacatgataagatacattgatgagtttggacaaaccacaactagaatgcagtgaaaaaaatgctttatttgtgaaatttgtgatgctattgctttatttgtaaccattataagctgcaataaacaagttaacaacaacaattgcattcattttatgtttcaggttcagggggaggtgtgggaggttttttaaagcaagtaaaacctctacaaatgtggtcctgcaggaacttgtttatttgaaaatcaattcacaaaatccgagtagttattttgcctcccccttcccatttaacagaatacaccaatctctccccacgcacagctttaaacatttggataccattagatatagacatggttttagattccacattccaaacagtttcagagcgagccaatctggggtcagtgatagataaaaatccatcgggatagtcttttaaagcgctttcacagtccaactgctgcggatgcgactccggagtctggatcacggtcatctggaagaagaacgatgggaatcataatccgaaaacggtatcggacgattgtgtctcatcaaacccacaagcagccgctgtctgcgtcgctccgtgcgactgctgtttatgggatcagggtccacagtgtcctgaagcatgattttaatagcccttaacatcaactttctggtgcgatgcgcgcagcaacgcattctgatttcactcaaatctttgcagtaggtacaacacattattacaatattgtttaataaaccataattaaaagcgctccagccaaaactcatatctgatataatcgcccctgcatgaccatcataccaaagtttaatataaattaaatgacgttccctcaaaaacacactacccacatacatgatctcttttggcatgtgcatattaacaatctgtctgtaccatggacaacgttggttaatcatgcaacccaatataaccttccggaaccacactgccaacaccgctcccccagccatgcattgaagtgaaccctgctgattacaatgacaatgaagaacccaattctctcgaccgtgaatcacttgagaatgaaaaatatctatagtggcacaacatagacataaatgcatgcatcttctcataatttttaactcctcaggatttagaaacatatcccagggaataggaagctcttgcagaacagtaaagctggcagaacaaggaagaccacgaacacaacttacactatgcatagtcatagtatcacaatctggcaacagcgggtggtcttcagtcatagaagctcgggtttcattttcctcacaacgtggtaactgggctctggtgtaagggtgatgtctggcgcatgatgtcgagcgtgcgcgcaaccttgtcataatggagttgcttcctgacattctcgtattttgtatagcaaaacgcggccctggcagaacacactcttcttcgccttctatcctgccgcttagcgtgttccgtgtgatagttcaagtacaaccacactcttaagttggtcaaaagaatgctggcttcagttgtaatcaaaactccatcgcatctaatcgttctgaggaaatcatccaagcaatgcaactggattgtgtttcaagcaggagaggagagggaagagacggaagaaccatgttaatttttattccaaacgatctcgcagtacttcaaattgtagatcgcgcagatggcatctctcgcccccactgtgttggtgaaaaagcacagctagatcaaaagaaatgcgattttcaaggtgctcaacggtggcttccagcaaagcctccacgcgcacatccaagaacaaaagaataccaaaagaaggagcattttctaactcctcaatcatcatattacattcctgcaccattcccagataattttcagctttccagccttgaattattcgtgtcagttcttgtggtaaatccaatccacacattacaaacaggtcccggagggcgccctccaccaccattcttaaacacaccctcataatgacaaaatatcttgctcctgtgtcacctgtagcgaattgagaatggcaacatcaattgacatgcccttggctctaagttcttctttaagttctagttgtaaaaactctctcatattatcaccaaactgcttagccagaagccccccgggaacaagagcaggggacgctacagtgcagtacaagcgcagacctccccaattggctccagcaaaaacaagattggaataagcatattgggaaccgccagtaatatcatcgaagttgctggaaatataatcaggcagagtttcttgtaaaaattgaataaaagaaaaatttgccaaaaaaacattcaaaacctctgggatgcaaatgcaataggttaccgcgctgcgctccaacattgttagttttgaattagtctgcaaaaataaaaaaaaaaacaagcgtcatatcatagtagcctgacgaacagatggataaatcagtctttccatcacaagacaagccacagggtctccagctcgaccctcgtaaaacctgtcatcatgattaaacaacagcaccgaaagttcctcgcggtgaccagcatgaataattcttgatgaagcatacaatccagacatgttagcatcagttaacgagaaaaaacagccaacatagcctttgggtataattatgcttaatcgtaagtatagcaaagccacccctcgcggatacaaagtaaaaggcacaggagaataaaaaatataattatttctctgctgctgttcaggcaacgtcgcccccggtccctctaaatacacatacaaagcctcatcagccatggcttaccagacaaagtacagcgggcacacaaagcacaagctctaaagtgactctccaacctctccacaatatatatatacacaagccctaaactgacgtaatgggagtaaagtgtaaaaaatcccgccaaacccaacacacaccccgaaactgcgtcaccagggaaaagtacagtttcacttccgcaatcccaacaggcgtaacttcctctttctcacggtacgtgatatcccactaacttgcaacgtcattttcccacggtcgcaccgccccttttagccgttaaccccacagccaatcaccacacgatccacactttttaaaatcacctcatttacatattggcaccattccatctataaggtatattatatagataga

SEQ ID NO: 2 - skipped

SEQ ID NO: 3 - protein, 19 aa, Artificial Sequence
  Heavy chain leader sequence
MDWTWRILFLVAAATGAHS

SEQ ID NO: 4 - protein, 126 aa, Artificial Sequence
  anti-CD40 VH chain amino acid sequence
QVQLVQSGAEVKKPGASVKVSCKASGYTFTGYYMHWVRQAPGQGLEWMGWINPDSGGTNYAQKFQGRVTMTRDTSISTAYMELNRLRSDDTAVYYCARDQPLGYCTNGVCSYFDYWGQGTLVTVSS

SEQ ID NO: 5 - protein, 326 aa, Artificial Sequence
  antibody constant heavy chain amino acid sequence
ASTKGPSVFPLAPCSRSTSESTAALGCLVKDYFPEPVTVSWNSGALTSGVHTFPAVLQSSGLYSLSSVVTVPSSNFGTQTYTCNVDHKPSNTKVDKTVERKCCVECPPCPAPPVAGPSVFLFPPKPKDTLMISRTPEVTCVVVDVSHEDPEVQFNWYVDGVEVHNAKTKPREEQFNSTFRVVSVLTVVHQDWLNGKEYKCKVSNKGLPAPIEKTISKTKGQPREPQVYTLPPSREEMTKNQVSLTCLVKGFYPSDIAVEWESNGQPENNYKTTPPMLDSDGSFFLYSKLTVDKSRWQQGNVFSCSVMHEALHNHYTQKSLSLSPGK

SEQ ID NO: 6 - skipped

SEQ ID NO: 7 - protein, 19 aa, Artificial Sequence
  Light chain leader sequence
RLPAQLLGLLLLWFPGSRC

SEQ ID NO: 8 - protein, 107 aa, Artificial Sequence
  anti-CD40 VL chain amino acid sequence
DIQMTQSPSSVSASVGDRVTITCRASQGIYSWLAWYQQKPGKAPNLLIYTASTLQSGVPSRFSGSGSGTDFTLTISSLQPEDFATYYCQQANIFPLTFGGGTKVEIK

SEQ ID NO: 9 - protein, 107 aa, Artificial Sequence [sequence omitted]

SEQ ID NO: 10 - DNA, 192 bp, Artificial Sequence
  Poly Adenylation sequence
cagacatgataagatacattgatgagtttggacaaaccacaactagaatgcagtgaaaaaaatgctttatttgtgaaatttgtgatgctattgctttatttgtaaccattataagctgcaataaacaagttaacaacaacaattgcattcattttatgtttcaggttcagggggaggtgtgggaggtttttt

SEQ ID NO: 11 - DNA, 2468 bp, Artificial Sequence
  NG-350 transgene cassette nucleic acid sequence
gcgatcgccaggcccaccatggactggacctggaggatcctcttcttggtggcagcagccacaggagcccactcccaggtgcagctggtgcagtctggggctgaggtgaagaagcctggggcctcagtgaaggtctcctgcaaggcttctggatacaccttcaccggctactatatgcactgggtgcgacaggcccctggacaagggcttgagtggatgggatggatcaaccctgacagtggtggcacaaactatgcacagaagtttcagggcagggtcaccatgaccagggacacgtccatcagcacagcctacatggagctgaacaggctgagatctgacgacacggccgtgtattactgtgcgagagatcagcccctaggatattgtactaatggtgtatgctcctactttgactactggggccagggaaccctggtcaccgtctcctcagcctccaccaagggcccatcggtcttccccctggcgccctgctccaggagcacctccgagagcacagcggccctgggctgcctggtcaaggactacttccccgaaccggtgacggtgtcgtggaactcaggcgctctgaccagcggcgtgcacaccttcccagctgtcctacagtcctcaggactctactccctcagcagcgtggtgaccgtgccctccagcaacttcggcacccagacctacacctgcaacgtagatcacaagcccagcaacaccaaggtggacaagacagttgagcgcaaatgttgtgtcgagtgcccaccgtgcccagcaccacctgtggcaggaccgtcagtcttcctcttccccccaaaacccaaggacaccctcatgatctcccggacccctgaggtcacgtgcgtggtggtggacgtgagccacgaagaccccgaggtccagttcaactggtacgtggacggcgtggaggtgcataatgccaagacaaagccacgggaggagcagttcaacagcacgttccgtgtggtcagcgtcctcaccgttgtgcaccaggactggctgaacggcaaggagtacaagtgcaaggtctccaacaaaggcctcccagcccccatcgagaaaaccatctccaaaaccaaagggcagccccgagaaccacaggtgtacaccctgcccccatcccgggaggagatgaccaagaaccaggtcagcctgacctgcctggtcaaaggcttctaccccagcgacatcgccgtggagtgggagagcaatgggcagccggagaacaactacaagaccacacctcccatgctggactccgacggctccttcttcctctacagcaagctcaccgtggacaagagcaggtggcagcaggggaacgtcttctcatgctccgtgatgcatgaggctctgcacaaccactacacgcagaagagcctctccctgtctccgggtaaaggaagcggagctactaacttcagcctgctgaagcaggctggagacgtggaggagaaccctggacctaggctccctgctcagctcctggggctcctgctgctctggttcccaggttccagatgcgacatccagatgacccagtctccatcttccgtgtctgcatctgtaggagacagagtcaccatcacttgtcgggcgagtcagggtatttacagctggttagcctggtatcagcagaaaccagggaaagcccctaacctcctgatctatactgcatccactttacaaagtggggtcccatcaaggttcagcggcagtggatctgggacagatttcactctcaccatcagcagcctgcaacctgaagattttgcaacttactattgtcaacaggctaacattttcccgctcactttcggcggagggaccaaggtggagatcaaacgaactgtggctgcaccatctgtcttcatcttcccgccatctgatgagcagttgaaatctggaactgcctctgttgtgtgcctgctgaataacttctatcccagagaggccaaagtacagtggaaggtggataacgccctccaatcgggtaactcccaggagagtgtcacagagcaggacagcaaggacagcacctacagcctcagcagcaccctgacgctgagcaaagcagactacgagaaacacaaagtctacgcctgcgaagtcacccatcagggcctgagctcgcccgtcacaaagagcttcaacaggggagagtgttaggctagcttgactgactgagatacagcgtaccttcagctcacagacatgataagatacattgatgagtttggacaaaccacaactagaatgcagtgaaaaaaatgctttatttgtgaaatttgtgatgctattgctttatttgtaaccattataagctgcaataaacaagttaacaacaacaattgcattcattttatgtttcaggttcagggggaggtgtgggaggttttttaaagcaagtaaaacctctacaaatgtggtcctgcagg

SEQ ID NO: 12 - DNA, 2468 bp, Artificial Sequence
  NG-350A transgene cassette nucleic acid sequence
gcgatcgccaggcccaccatggactggacctggcgcatcctgttcttggtggcagctgctacgggagctcattcccaggtgcagctggtgcaatccggcgctgaggtgaagaaacccggggcttcagtcaaagtcagctgcaaggctagcggctacacctttactggctattacatgcactgggtgaggcaggctccgggacagggtctggaatggatgggatggatcaatccggacagcggcgggaccaattacgcacaaaagttccaaggccgcgtgacgatgacccgggacacttcgatctcaaccgcctacatggagctgaaccgcctgaggtcggatgacaccgctgtgtactactgcgctcgcgaccaacccctggggtactgcaccaacggagtgtgttcatacttcgactactggggccaaggcacgctggtcactgtgtcatcggcgtccactaagggcccgtcggtcttcccactagctccgtgctcgcggtcgacttcggaatcaactgcggcactcggatgccttgtcaaggactacttcccagaacccgtgaccgtctcgtggaactcaggcgccctgacgagcggtgtccacactttcccggcggtgctgcagtcatcggggctatacagcctgagcagcgtggttactgtgccgtcatcaaacttcgggacccagacttacacttgcaatgtggaccacaagccgtcaaataccaaagtggacaagactgtggaacgcaaatgttgcgtggaatgccctccgtgcccggcccccccagtcgctggcccatccgtgttcctcttccctccgaagccaaaagacactctgatgatttcgagaactccggaggtcacttgcgtggtggtcgacgtgtcgcacgaggatccagaggtgcagttcaactggtacgtggatggagtggaggtgcacaatgccaagaccaagccgcgcgaagaacaattcaactccacctttcgggtcgtgtccgtgctgaccgtggtacaccaagactggctgaacggaaaggagtacaaatgcaaggtgagcaacaaggggctgccggctccaatcgaaaagaccatctcaaagactaaggggcaacctcgcgagccacaggtgtataccctgcctccaagcagggaggaaatgaccaaaaaccaggtgagcctgacctgtctggtgaagggcttttaccccagcgacatcgccgtcgagtgggaaagcaacggacaacccgagaacaactacaagaccactccgcccatgctggactccgacgggtcatttttcctgtactcaaagctgactgtggacaagtcccggtggcagcaaggtaacgtgttctcctgctcggtgatgcacgaagctttgcacaaccactacactcaaaagtcactttccttgtcaccgggcaaggggtcgggcgccactaacttttccttgctcaagcaggcgggcgatgtggaggagaatccgggcccgcgcctcccggcgcaactgctgggcctcctcctcctctggtttcccggctcccgctgtgacatccagatgactcagtcgcccagctccgtgtccgcatcggtgggggacagagtcaccatcacctgcagagcttcacaagggatctattcctggctggcgtggtatcagcagaagcctggaaaggcccccaacctcctgatttacaccgcatcgactctccagtcaggcgtgccatcccggttctcagggtccggctccggaaccgacttcactctgactatcagctccctgcaaccagaagatttcgctacctactactgccagcaggcaaacatctttccgctaactttcggcggaggcacgaaggtggagatcaagagaaccgtggcggccccttccgtcttcatcttcccaccgtcagacgaacaactcaaatccggtaccgcctccgtcgtgtgcctgctcaataacttctatccacgcgaggccaaggtccagtggaaagtggataacgccctgcagtccggaaacagccaggagtcagtgaccgaacaggattccaaggacagcacttactcgctctcaagcaccctcaccctgtcgaaggcggattacgagaagcacaaagtctacgcctgcgaagtgactcatcaaggactctcatcaccggtaactaagagcttcaatcgcggagaatgctaggctagcttgactgactgagatacagcgtaccttcagctcacagacatgataagatacattgatgagtttggacaaaccacaactagaatgcagtgaaaaaaatgctttatttgtgaaatttgtgatgctattgctttatttgtaaccattataagctgcaataaacaagttaacaacaacaattgcattcattttatgtttcaggttcagggggaggtgtgggaggttttttaaagcaagtaaaacctctacaaatgtggtcctgcagg

SEQ ID NO: 13 - DNA, 34794 bp, Artificial Sequence
  NG-350 Virus Genome
tctatctatataatataccttatagatggaatggtgccaatatgtaaatgaggtgattttaaaaagtgtggatcgtgtggtgattggctgtggggttaacggctaaaaggggcggtgcgaccgtgggaaaatgacgttttgtgggggtggagtttttttgcaagttgtcgcgggaaatgtgacgcataaaaaggcttttttctcacggaactacttagttttcccacggtatttaacaggaaatgaggtagttttgaccggatgcaagtgaaaattgttgattttcgcgcgaaaactgaatgaggaagtgtttttctgaataatgtggtatttatggcagggtggagtatttgttcagggccaggtagactttgacccattacgtggaggtttcgattaccgtgttttttacctgaatttccgcgtaccgtgtcaaagtcttctgtttttacgtaggtgtcagctgatcgctagggtatttatacctcagggtttgtgtcaagaggccactcttgagtgccagcgagaagagttttctcctctgcgccggcagtttaataataaaaaaatgagagatttgcgatttctgcctcaggaaataatctctgctgagactggaaatgaaatattggagcttgtggtgcacgccctgatgggagacgatccggagccacctgtgcagctttttgagcctcctacgcttcaggaactgtatgatttagaggtagagggatcggaggattctaatgaggaagctgtaaatggcttttttaccgattctatgcttttagctgctaatgaagggttagaattagatccgcctttggacacttttgatactccaggggtaattgtggaaagcggtacaggtgtaagaaaattacctgatttgagttccgtggactgtgatttgcactgctatgaagacgggtttcctccgagtgatgaggaggaccatgaaaaggagcagtccatgcagactgcagcgggtgagggagtgaaggctgccaatgttggttttcagttggattgcccggagcttcctggacatggctgtaagtcttgtgaatttcacaggaaaaatactggagtaaaggaactgttatgttcgctttgttatatgagaacgcactgccactttatttacagtaagtgtgtttaagttaaaatttaaaggaatatgctgtttttcacatgtatattgagtgtgagttttgtgcttcttattataggtcctgtgtctgatgctgatgaatcaccatctcctgattctactacctcacctcctgagattcaagcacctgttcctgtggacgtgcgcaagcccattcctgtgaagcttaagcctgggaaacgtccagcagtggaaaaacttgaggacttgttacagggtggggacggacctttggacttgagtacacggaaacgtccaagacaataagtgttccatatccgtgtttacttaaggtgacgtcaatatttgtgtgacagtgcaatgtaataaaaatatgttaactgttcactggtttttattgctttttgggcggggactcaggtatataagtagaagcagacctgtgtggttagctcataggagctggctttcatccatggaggtttgggccattttggaagaccttaggaagactaggcaactgttagagaacgcttcggacggagtctccggtttttggagattctggttcgctagtgaattagctagggtagtttttaggataaaacaggactataaacaagaatttgaaaagttgttggtagattgcccaggactttttgaagctcttaatttgggccatcaggttcactttaaagaaaaagttttatcagttttagacttttcaaccccaggtagaactgctgctgctgtggcttttcttacttttatattagataaatggatcccgcagactcatttcagcaggggatacgttttggatttcatagccacagcattgtggagaacatggaaggttcgcaagatgaggacaatcttaggttactggccagtgcagcctttgggtgtagcgggaatcctgaggcatccaccggtcatgccagcggttctggaggaggaacagcaagaggacaacccgagagccggcctggaccctccagtggaggaggcggagtagctgacttgtctcctgaactgcaacgggtgcttactggatctacgtccactggacgggataggggcgttaagagggagagggcatctagtggtactgatgctagatctgagttggctttaagtttaatgagtcgcagacgtcctgaaaccatttggtggcatgaggttcagaaagagggaagggatgaagtttctgtattgcaggagaaatattcactggaacaggtgaaaacatgttggttggagcctgaggatgattgggaggtggccattaaaaattatgccaagatagctttgaggcctgataaacagtataagattactagacggattaatatccggaatgcttgttacatatctggaaatggggctgaggtggtaatagatactcaagacaaggcagttattagatgctgcatgatggatatgtggcctggggtagtcggtatggaagcagtaacttttgtaaatgttaagtttaggggagatggttataatggaatagtgtttatggccaataccaaacttatattgcatggttgtagcttttttggtttcaacaatacctgtgtagatgcctggggacaggttagtgtacggggatgtagtttctatgcgtgttggattgccacagctggcagaaccaagagtcaattgtctctgaagaaatgcatatttcaaagatgtaacctgggcattctgaatgaaggcgaagcaagggtccgccactgcgcttctacagatactggatgttttattttgattaagggaaatgccagcgtaaagcataacatgatttgcggtgcttccgatgagaggccttatcaaatgctcacttgtgctggtgggcattgtaatatgctggctactgtgcatattgtttcccatcaacgcaaaaaatggcctgtttttgatcacaatgtgatgacgaagtgtaccatgcatgcaggtgggcgtagaggaatgtttatgccttaccagtgtaacatgaatcatgtgaaagtgttgttggaaccagatgccttttccagaatgagcctaacaggaatttttgacatgaacatgcaaatctggaagatcctgaggtatgatgatacgagatcgagggtacgcgcatgcgaatgcggaggcaagcatgccaggttccagccggtgtgtgtagatgtgactgaagatctcagaccggatcatttggttattgcccgcactggagcagagttcggatccagtggagaagaaactgactaaggtgagtattgggaaaactttggggtgggattttcagatggacagattgagtaaaaatttgttttttctgtcttgcagctgtcatgagtggaaacgcttcttttaaggggggagtcttcagcccttatctgacagggcgtctcccatcctgggcaggagttcgtcagaatgttatgggatctactgtggatggaagacccgtccaacccgccaattcttcaacgctgacctatgctactttaagttcttcacctttggacgcagctgcagctgccgccgccgcttctgttgccgctaacactgtgcttggaatgggttactatggaagcatcatggctaattccacttcctctaataacccttctaccctgactcaggacaagttacttgtccttttggcccagctggaggctttgacccaacgtctgggtgaactttctcagcaggtggtcgagttgcgagtacaaactgagtctgctgtcggcacggcaaagtctaaataaaaaaatcccagaatcaatgaataaataaacaagcttgttgttgatttaaaatcaagtgtttttatttcatttttcgcgcacggtatgccctagaccaccgatctctatcattgagaactcggtggattttttccaggatcctatagaggtgggattgaatgtttagatacatgggcattaggccgtctttggggtggagatagctccattgaagggattcatgctccggggtagtgttgtaaatcacccagtcataacaaggtcgcagtgcatggtgttgcacaatatcttttagaagtaggctgattgccacagataagcccttggtgtaggtgtttacaaaccggttgagctgggatgggtgcattcggggtgaaattatgtgcattttggattggatttttaagttggcaatattgccgccaagatcccgtcttgggttcatgttatgaaggaccaccaagacggtgtatccggtacatttaggaaatttatcgtgcagcttggatggaaaagcgtggaaaaatttggagacacccttgtgtcctccaagattttccatgcactcatccatgataatagcaatggggccgtgggcagcggcgcgggcaaacacgttccgtgggtctgacacatcatagttatgttcctgagttaaatcatcataagccattttaatgaatttggggcggagagtaccagattggggtatgaatgttccttcgggccccggagcatagttcccctcacagatttgcatttcccaagctttcagttccgagggtggaatcatgtccacctggggggctatgaaaaacaccgtttctggggcgggggtgattaattgtgatgatagcaaatttctgagcaattgagatttgccacatccggtggggccataaatgattccgattacgggttgcaggtggtagtttagggaacggcaactgccgtcttctcgaagcaagggggccacctcgttcatcatttcccttacatgcatattttcccgcaccaaatccattaggaggcgctctcctcctagtgatagaagttcttgtagtgaggaaaagtttttcagcggtttcagaccgtcagccatgggcattttggagagagtttgctgcaaaagttctagtctgttccacagttcagtgatgtgttctatggcatctcgatccagcagacctcctcgtttcgcgggtttggacggctcctggaatagggtatgagacgatgggcgtccagcgctgccagggttcggtccttccagggtctcagtgttcgagtcagggttgtttccgtcacagtgaaggggtgtgcgcctgcttgggcgcttgccagggtgcgcttcagactcatcctgctggtcgaaaacttctgtcgcttggcgccctgtatgtcggccaagtagcagtttaccatgagttcgtagttgagcgcctcggctgcgtggcctttggcgcggagcttacctttggaagttttcttgcataccgggcagtataggcatttcagcgcatacaacttgggcgcaaggaaaacggattctggggagtatgcatctgcgccgcaggaggcgcaaacagtttcacattccaccagccaggttaaatccggttcattggggtcaaaaacaagttttccgccatattttttgatgcgtttcttacctttggtctccatgagttcgtgtcctcgttgagtgacaaacaggctgtccgtgtccccgtagactgattttacaggcctcttctccagtggagtgcctcggtcttcttcgtacaggaactctgaccactctgatacaaaggcgcgcgtccaggccagcacaaaggaggctatgtgggaggggtagcgatcgttgtcaaccagggggtccaccttttccaaagtatgcaaacacatgtcaccctcttcaacatccaggaatgtgattggcttgtaggtgtatttcacgtgacctggggtccccgctgggggggtataaaagggggcggttctttgctcttcctcactgtcttccggatcgctgtccaggaacgtcagctgttggggtaggtattccctctcgaaggcgggcatgacctctgcactcaggttgtcagtttctaagaacgaggaggatttgatattgacagtgccggttgagatgcctttcatgaggttttcgtccatctggtcagaaaacacaatttttttattgtcaagtttggtggcaaatgatccatacagggcgttggataaaagtttggcaatggatcgcatggtttggttcttttccttgtccgcgcgctctttggcggcgatgttgagttggacatactcgcgtgccaggcacttccattcggggaagatagttgttaattcatctggcacgattctcacttgccaccctcgattatgcaaggtaattaaatccacactggtggccacctcgcctcgaaggggttcattggtccaacagagcctacctcctttcctagaacagaaagggggaagtgggtctagcataagttcatcgggagggtctgcatccatggtaaagattcccggaagtaaatccttatcaaaatagctgatgggagtggggtcatctaaggccatttgccattctcgagctgccagtgcgcgctcatatgggttaaggggactgccccatggcatgggatgggtgagtgcagaggcatacatgccacagatgtcatagacgtagatgggatcctcaaagatgcctatgtaggttggatagcatcgcccccctctgatacttgctcgcacatagtcatatagttcatgtgatggcgctagcagccccggacccaagttggtgcgattgggtttttctgttctgtagacgatctggcgaaagatggcgtgagaattggaagagatggtgggtctttgaaaaatgttgaaatgggcatgaggtagacctacagagtctctgacaaagtgggcataagattcttgaagcttggttaccagttcggcggtgacaagtacgtctagggcgcagtagtcaagtgtttcttgaatgatgtcataacctggttggtttttcttttcccacagttcgcggttgagaaggtattcttcgcgatccttccagtactcttctagcggaaacccgtctttgtctgcacggtaagatcctagcatgtagaactgattaactgccttgtaagggcagcagcccttctctacgggtagagagtatgcttgagcagcttttcgtagcgaagcgtgagtaagggcaaaggtgtctctgaccatgactttgaggaattggtatttgaagtcgatgtcgtcacaggctccctgttcccagagttggaagtctacccgtttcttgtaggcggggttgggcaaagcgaaagtaacatcattgaagagaatcttgccggccctgggcatgaaattgcgagtgatgcgaaaaggctgtggtacttccgctcggttattgataacctgggcagctaggacgatctcgtcgaaaccgttgatgttgtgtcctacgatgtataattctatgaaacgcggcgtgcctctgacgtgaggtagcttactgagctcatcaaaggttaggtctgtggggtcagataaggcgtagtgttcgagagcccattcgtgcaggtgaggattcgctttaaggaaggaggaccagaggtccactgccagtgctgtttgtaactggtcccggtactgacgaaaatgccgtccgactgccattttttctggggtgacgcaatagaaggtttgggggtcctgccgccagcgatcccacttgagttttatggcgaggtcataggcgatgttgacgagccgctggtctccagagagtttcatgaccagcatgaaggggattagctgcttgccaaaggaccccatccaggtgtaggtttccacatcgtaggtgagaaagagcctttctgtgcgaggatgagagccaatcgggaagaactggatctcctgccaccagttggaggaatggctgttgatgtgatggaagtagaactccctgcgacgcgccgagcattcatgcttgtgcttgtacagacggccgcagtagtcgcagcgttgcacgggttgtatctcgtgaatgagttgtacctggcttcccttgacgagaaatttcagtgggaagccgaggcctggcgattgtatctcgtgctttactatgttgtctgcatcggcctgttcatcttctgtctcgatggtggtcatgctgacgagccctcgcgggaggcaagtccagacctcggcgcggcaggggcggagctcgaggacgagagcgcgcaggctggagctgtccagggtcctgagacgctgcggactcaggttagtaggcagtgtcaggagattaacttgcatgatcttttggagggcgtgcgggaggttcagatagtacttgatctcaacgggtccgttggtggagatgtcgatggcttgcagggttccgtgtcccttgggcgctaccaccgtgcccttgtttttcattttggacggcggtggctctgttgcttcttgcatgtttagaagcggtgtcgagggcgcgcaccgggcggcaggggcggctcgggacccggcggcatggctggcagtggtacgtcggcgccgcgcgcgggtaggttctggtactgcgccctgagaagactcgcatgcgcgacgacgcggcggttgacatcctggatctgacgcctctgggtgaaagctaccggccccgtgagcttgaacctgaaagagagttcaacagaatcaatctcggtatcgttgacggcggcttgcctaaggatttcttgcacgtcaccagagttgtcctggtaggcgatctccgccatgaactgctcgatctcttcctcttgaagatctccgcggcccgctctctcgacggtggccgcgaggtcgttggagatgcgcccaatgagttgagagaatgcattcatgcccgcctcgttccagacgcggctgtagaccacggcccccacgggatctctcgcgcgcatgaccacctgggcgaggttgagctccacgtggcgggtgaagaccgcatagttgcataggcgctggaaaaggtagttgagtgtggtggcgatgtgctcggtgacgaagaaatacatgatccatcgtctcagcggcatctcgctgacatcgcccagagcttccaagcgctccatggcctcgtagaagtccacggcaaaattaaaaaactgggagtttcgcgcggacacggtcaactcctcttccagaagacggataagttcggcgatggtggtgcgcacctcgcgctcgaaagcccctgggatttcttcctcaatctcttcttcttccactaacatctcttcctcttcaggtggggctgcaggaggagggggaacgcggcgacgccggcggcgcacgggcagacggtcgatgaatctttcaatgacctctccgcggcggcggcgcatggtttcagtgacggcgcggccgttctcgcgcggtcgcagagtaaaaacaccgccgcgcatctccttaaagtggtgactgggaggttctccgtttgggagggagagggcgctgattatacattttattaattggcccgtagggactgcacgcagagatctgatcgtgtcaagatccacgggatctgaaaacctttcgacgaaagcgtctaaccagtcacagtcacaaggtaggctgagtacggcttcttgtgggcgggggtggttatgtgttcggtctgggtcttctgtttcttcttcatctcgggaaggtgagacgatgctgctggtgatgaaattaaagtaggcagttctaagacggcggatggtggcgaggagcaccaggtctttgggtccggcttgctggatacgcaggcgattggccattccccaagcattatcctgacatctagcaagatctttgtagtagtcttgcatgagccgttctacgggcacttcttcctcacccgttctgccatgcatacgtgtgagtccaaatccgcgcattggttgtaccagtgccaagtcagctacgactctttcggcgaggatggcttgctgtacttgggtaagggtggcttgaaagtcatcaaaatccacaaagcggtggtaagctcctgtattaatggtgtaagcacagttggccatgactgaccagttaactgtctggtgaccagggcgcacgagctcggtgtatttaaggcgcgaataggcgcgggtgtcaaagatgtaatcgttgcaggtgcgcaccagatactggtaccctataagaaaatgcggcggtggttggcggtagagaggccatcgttctgtagctggagcgccaggggcgaggtcttccaacataaggcggtgatagccgtagatgtacctggacatccaggtgattcctgcggcggtagtagaagcccgaggaaactcgcgtacgcggttccaaatgttgcgtagcggcatgaagtagttcattgtaggcacggtttgaccagtgaggcgcgcgcagtcattgatgctctatagacacggagaaaatgaaagcgttcagcgactcgactccgtagcctggaggaacgtgaacgggttgggtcgcggtgtaccccggttcgagacttgtactcgagccggccggagccgcggctaacgtggtattggcactcccgtctcgacccagcctacaaaaatccaggatacggaatcgagtcgttttgctggtttccgaatggcagggaagtgagtcctattttttttttttgccgctcagatgcatcccgtgctgcgacagatgcgcccccaacaacagcccccctcgcagcagcagcagcagcaatcacaaaaggctgtccctgcaactactgcaactgccgccgtgagcggtgcgggacagcccgcctatgatctggacttggaagagggcgaaggactggcacgtctaggtgcgccttcacccgagcggcatccgcgagttcaactgaaaaaagattctcgcgaggcgtatgtgccccaacagaacctatttagagacagaagcggcgaggagccggaggagatgcgagcttcccgctttaacgcgggtcgtgagctgcgtcacggtttggaccgaagacgagtgttgcgggacgaggatttcgaagttgatgaaatgacagggatcagtcctgccagggcacacgtggctgcagccaaccttgtatcggcttacgagcagacagtaaaggaagagcgtaacttccaaaagtcttttaataatcatgtgcgaaccctgattgcccgcgaagaagttacccttggtttgatgcatttgtgggatttgatggaagctatcattcagaaccctactagcaaacctctgaccgcccagctgtttctggtggtgcaacacagcagagacaatgaggctttcagagaggcgctgctgaacatcaccgaacccgaggggagatggttgtatgatcttatcaacattctacagagtatcatagtgcaggagcggagcctgggcctggccgagaaggtggctgccatcaattactcggttttgagcttgggaaaatattacgctcgcaaaatctacaagactccatacgttcccatagacaaggaggtgaagatagatgggttctacatgcgcatgacgctcaaggtcttgaccctgagcgatgatcttggggtgtatcgcaatgacagaatgcatcgcgcggttagcgccagcaggaggcgcgagttaagcgacagggaactgatgcacagtttgcaaagagctctgactggagctggaaccgagggtgagaattacttcgacatgggagctgacttgcagtggcagcctagtcgcagggctctgagcgccgcgacggcaggatgtgagcttccttacatagaagaggcggatgaaggcgaggaggaagagggcgagtacttggaagactgatggcacaacccgtgttttttgctagatggaacagcaagcaccggatcccgcaatgcgggcggcgctgcagagccagccgtccggcattaactcctcggacgattggacccaggccatgcaacgtatcatggcgttgacgactcgcaaccccgaagcctttagacagcaaccccaggccaaccgtctatcggccatcatggaagctgtagtgccttcccgctctaatcccactcatgagaaggtcctggccatcgtgaacgcgttggtggagaacaaagctattcgtccagatgaggccggactggtatacaacgctctcttagaacgcgtggctcgctacaacagtagcaatgtgcaaaccaatttggaccgtatgataacagatgtacgcgaagccgtgtctcagcgcgaaaggttccagcgtgatgccaacctgggttcgctggtggcgttaaatgctttcttgagtactcagcctgctaatgtgccgcgtggtcaacaggattatactaactttttaagtgctttgagactgatggtatcagaagtacctcagagcgaagtgtatcagtccggtcctgattacttctttcagactagcagacagggcttgcagacggtaaatctgagccaagcttttaaaaaccttaaaggtttgtggggagtgcatgccccggtaggagaaagagcaaccgtgtctagcttgttaactccgaactcccgcctattattactgttggtagctcctttcaccgacagcggtagcatcgaccgtaattcctatttgggttacctactaaacctgtatcgcgaagccatagggcaaagtcaggtggacgagcagacctatcaagaaattacccaagtcagtcgcgctttgggacaggaagacactggcagtttggaagccactctgaacttcttgcttaccaatcggtctcaaaagatccctcctcaatatgctcttactgcggaggaggagaggatccttagatatgtgcagcagagcgtgggattgtttctgatgcaagagggggcaactccgactgcagcactggacatgacagcgcgaaatatggagcccagcatgtatgccagtaaccgacctttcattaacaaactgctggactacttgcacagagctgccgctatgaactctgattatttcaccaatgccatcttaaacccgcactggctgcccccacctggtttctacacgggcgaatatgacatgcccgaccctaatgacggatttctgtgggacgacgtggacagcgatgttttttcacctctttctgatcatcgcacgtggaaaaaggaaggcggcgatagaatgcattcttctgcatcgctgtccggggtcatgggtgctaccgcggctgagcccgagtctgcaagtccttttcctagtctacccttttctctacacagtgtacgtagcagcgaagtgggtagaataagtcgcccgagtttaatgggcgaagaggagtatctaaacgattccttgctcagaccggcaagagaaaaaaatttcccaaacaatggaatagaaagtttggtggataaaatgagtagatggaagacttatgctcaggatcacagagacgagcctgggatcatggggattacaagtagagcgagccgtagacgccagcgccatgacagacagaggggtcttgtgtgggacgatgaggattcggccgatgatagcagcgtgctggacttgggtgggagaggaaggggcaacccgtttgctcatttgcgccctcgcttgggtggtatgttgtaaaaaaaaataaaaaaaaaactcaccaaggccatggcgacgagcgtacgttcgttcttctttattatctgtgtctagtataatgaggcgagtcgtgctaggcggagcggtggtgtatccggagggtcctcctccttcgtacgagagcgtgatgcagcagcagcaggcgacggcggtgatgcaatccccactggaggctccctttgtgcctccgcgatacctggcacctacggagggcagaaacagcattcgttattcggaactggcacctcagtacgataccaccaggttgtatctggtggacaacaagtcggcggacattgcttctctgaactatcagaatgaccacagcaacttcttgaccacggtggtgcaaaacaatgactttacccctacggaagccagcacccagaccattaactttgatgaacgatcgcggtggggcggtcagctaaagaccatcatgcatactaacatgccaaacgtgaacgagtatatgtttagtaacaagttcaaagcgcgtgtgatggtgtccagaaaacctcccgacggtgctgcagttggggatacttatgatcacaagcaggatattttgaaatatgagtggttcgagtttactttgccagaaggcaacttttcagttactatgactattgatttgatgaacaatgccatcatagataattacttgaaagtgggtagacagaatggagtgcttgaaagtgacattggtgttaagttcgacaccaggaacttcaagctgggatgggatcccgaaaccaagttgatcatgcctggagtgtatacgtatgaagccttccatcctgacattgtcttactgcctggctgcggagtggattttaccgagagtcgtttgagcaaccttcttggtatcagaaaaaaacagccatttcaagagggttttaagattttgtatgaagatttagaaggtggtaatattccggccctcttggatgtagatgcctatgagaacagtaagaaagaacaaaaagccaaaatagaagctgctacagctgctgcagaagctaaggcaaacatagttgccagcgactctacaagggttgctaacgctggagaggtcagaggagacaattttgcgccaacacctgttccgactgcagaatcattattggccgatgtgtctgaaggaacggacgtgaaactcactattcaacctgtagaaaaagatagtaagaatagaagctataatgtgttggaagacaaaatcaacacagcctatcgcagttggtatctttcgtacaattatggcgatcccgaaaaaggagtgcgttcctggacattgctcaccacctcagatgtcacctgcggagcagagcaggtctactggtcgcttccagacatgatgaaggatcctgtcactttccgctccactagacaagtcagtaactaccctgtggtgggtgcagagcttatgcccgtcttctcaaagagcttctacaacgaacaagctgtgtactcccagcagctccgccagtccacctcgcttacgcacgtcttcaaccgctttcctgagaaccagattttaatccgtccgccggcgcccaccattaccaccgtcagtgaaaacgttcctgctctcacagatcacgggaccctgccgttgcgcagcagtatccggggagtccaacgtgtgaccgttactgacgccagacgccgcacctgtccctacgtgtacaaggcactgggcatagtcgcaccgcgcgtcctttcaagccgcactttctaaaaaaaaaaaaaatgtccattcttatctcgcccagtaataacaccggttggggtctgcgcgctccaagcaagatgtacggaggcgcacgcaaacgttctacccaacatcctgtccgtgttcgcggacattttcgcgctccatggggcgccctcaagggccgcactcgcgttcgaaccaccgtcgatgatgtaatcgatcaggtggttgccgacgcccgtaattatactcctactgcgcctacatctactgtggatgcagttattgacagtgtagtggctgacgctcgcaactatgctcgacgtaagagccggcgaaggcgcattgccagacgccaccgagctaccactgccatgcgagccgcaagagctctgctacgaagagctagacgcgtggggcgaagagccatgcttagggcggccagacgtgcagcttcgggcgccagcgccggcaggtcccgcaggcaagcagccgctgtcgcagcggcgactattgccgacatggcccaatcgcgaagaggcaatgtatactgggtgcgtgacgctgccaccggtcaacgtgtacccgtgcgcacccgtccccctcgcacttagaagatactgagcagtctccgatgttgtgtcccagcggcgaggatgtccaagcgcaaatacaaggaagaaatgctgcaggttatcgcacctgaagtctacggccaaccgttgaaggatgaaaaaaaaccccgcaaaatcaagcgggttaaaaaggacaaaaaagaagaggaagatggcgatgatgggctggcggagtttgtgcgcgagtttgccccacggcgacgcgtgcaatggcgtgggcgcaaagttcgacatgtgttgagacctggaacttcggtggtctttacacccggcgagcgttcaagcgctacttttaagcgttcctatgatgaggtgtacggggatgatgatattcttgagcaggcggctgaccgattaggcgagtttgcttatggcaagcgtagtagaataacttccaaggatgagacagtgtcgatacccttggatcatggaaatcccacccctagtcttaaaccggtcactttgcagcaagtgttacccgtaactccgcgaacaggtgttaaacgcgaaggtgaagatttgtatcccactatgcaactgatggtacccaaacgccagaagttggaggacgttttggagaaagtaaaagtggatccagatattcaacctgaggttaaagtgagacccattaagcaggtagcgcctggtctgggggtacaaactgtagacattaagattcccactgaaagtatggaagtgcaaactgaacccgcaaagcctactgccacctccactgaagtgcaaacggatccatggatgcccatgcctattacaactgacgccgccggtcccactcgaagatcccgacgaaagtacggtccagcaagtctgttgatgcccaattatgttgtacacccatctattattcctactcctggttaccgaggcactcgctactatcgcagccgaaacagtacctcccgccgtcgccgcaagacacctgcaaatcgcagtcgtcgccgtagacgcacaagcaaaccgactcccggcgccctggtgcggcaagtgtaccgcaatggtagtgcggaacctttgacactgccgcgtgcgcgttaccatccgagtatcatcacttaatcaatgttgccgctgcctccttgcagatatggccctcacttgtcgccttcgcgttcccatcactggttaccgaggaagaaactcgcgccgtagaagagggatgttgggacgcggaatgcgacgctacaggcgacggcgtgctatccgcaagcaattgcggggtggttttttaccagccttaattccaattatcgctgctgcaattggcgcgataccaggcatagcttccgtggcggttcaggcctcgcaacgacattgacattggaaaaaaacgtataaataaaaaaaaaaaaatacaatggactctgacactcctggtcctgtgactatgttttcttagagatggaagacatcaatttttcatccttggctccgcgacacggcacgaagccgtacatgggcacctggagcgacatcggcacgagccaactgaacgggggcgccttcaattggagcagtatctggagcgggcttaaaaattttggctcaaccataaaaacatacgggaacaaagcttggaacagcagtacaggacaggcgcttagaaataaacttaaagaccagaacttccaacaaaaagtagtcgatgggatagcttccggcatcaatggagtggtagatttggctaaccaggctgtgcagaaaaagataaacagtcgtttggacccgccgccagcaaccccaggtgaaatgcaagtggaggaagaaattcctccgccagaaaaacgaggcgacaagcgtccgcgtcccgatttggaagagacgctggtgacgcgcgtagatgaaccgccttcttatgaggaagcaacgaagcttggaatgcccaccactagaccgatagccccaatggccaccggggtgatgaaaccttctcagttgcatcgacccgtcaccttggatttgccccctccccctgctgctactgctgtacccgcttctaagcctgtcgctgccccgaaaccagtcgccgtagccaggtcacgtcccgggggcgctcctcgtccaaatgcgcactggcaaaatactctgaacagcatcgtgggtctaggcgtgcaaagtgtaaaacgccgtcgctgcttttaattaaatatggagtagcgcttaacttgcctatctgtgtatatgtgtcattacacgccgtcacagcagcagaggaaaaaaggaagaggtcgtgcgtcgacgctgagttactttcaagatggccaccccatcgatgctgccccaatgggcatacatgcacatcgccggacaggatgcttcggagtacctgagtccgggtctggtgcagttcgcccgcgccacagacacctacttcaatctgggaaataagtttagaaatcccaccgtagcgccgacccacgatgtgaccaccgaccgtagccagcggctcatgttgcgcttcgtgcccgttgaccgggaggacaatacatactcttacaaagtgcggtacaccctggccgtgggcgacaacagagtgctggatatggccagcacgttctttgacattaggggtgtgttggacagaggtcccagtttcaaaccctattctggtacggcttacaactccctggctcctaaaggcgctccaaatacatctcagtggattgcagaaggtgtaaaaaatacaactggtgaggaacacgtaacagaagaggaaaccaatactactacttacacttttggcaatgctcctgtaaaagctgaagctgaaattacaaaagaaggactcccagtaggtttggaagtttcagatgaagaaagtaaaccgatttatgctgataaaacatatcagccagaacctcagctgggagatgaaacttggactgaccttgatggaaaaaccgaaaagtatggaggcagggctctcaaacccgatactaagatgaaaccatgctacgggtcctttgccaaacctactaatgtgaaaggcggtcaggcaaaacaaaaaacaacggagcagccaaatcagaaagtcgaatatgatatcgacatggagttttttgatgcggcatcgcagaaaacaaacttaagtcctaaaattgtcatgtatgcagaaaatgtaaatttggaaactccagacactcatgtagtgtacaaacctggaacagaagacacaagttccgaagctaatttgggacaacaatctatgcccaacagacccaactacattggcttcagagataactttattggacttatgtactataacagtactggtaacatgggggtgctggctggtcaagcgtctcagttaaatgcagtggttgacttgcaggacagaaacacagaactttcttaccaactcttgcttgactctctgggcgacagaaccagatactttagcatgtggaatcaggctgtggacagttatgatcctgatgtacgtgttattgaaaatcatggtgtggaagatgaacttcccaactactgttttccactggacggcataggtgttccaacaaccagttacaaatcaatagttccaaatggagacaatgcgcctaattggaaggaacctgaagtaaatggaacaagtgagatcggacagggtaatttgtttgccatggaaattaaccttcaagccaatctatggcgaagtttcctttattccaatgtggctctatatctcccagactcgtacaaatacaccccgtccaatgtcactcttccagaaaacaaaaacacctacgactacatgaacgggcgggtggtgccgccatctctagtagacacctatgtgaacattggtgccaggtggtctctggatgccatggacaatgtcaacccattcaaccaccaccgtaacgctggcttgcgttaccgatccatgcttctgggtaacggacgttatgtgcctttccacatacaagtgcctcaaaaattcttcgctgttaaaaacctgctgcttctcccaggctcctacacttatgagtggaactttaggaaggatgtgaacatggttctacagagttccctcggtaacgacctgcgggtagatggcgccagcatcagtttcacgagcatcaacctctatgctacttttttccccatggctcacaacaccgcttccacccttgaagccatgctgcggaatgacaccaatgatcagtcattcaacgactacctatctgcagctaacatgctctaccccattcctgccaatgcaaccaatattcccatttccattccttctcgcaactgggcggctttcagaggctggtcatttaccagactgaaaaccaaagaaactccctctttggggtctggatttgacccctactttgtctattctggttctattccctacctggatggtaccttctacctgaaccacacttttaagaaggtttccatcatgtttgactcttcagtgagctggcctggaaatgacaggttactatctcctaacgaatttgaaataaagcgcactgtggatggcgaaggctacaacgtagcccaatgcaacatgaccaaagactggttcttggtacagatgctcgccaactacaacatcggctatcagggcttctacattccagaaggatacaaagatcgcatgtattcatttttcagaaacttccagcccatgagcaggcaggtggttgatgaggtcaattacaaagacttcaaggccgtcgccataccctaccaacacaacaactctggctttgtgggttacatggctccgaccatgcgccaaggtcaaccctatcccgctaactatccctatccactcattggaacaactgccgtaaatagtgttacgcagaaaaagttcttgtgtgacagaaccatgtggcgcataccgttctcgagcaacttcatgtctatgggggcccttacagacttgggacagaatatgctctatgccaactcagctcatgctctggacatgacctttgaggtggatcccatggatgagcccaccctgctttatcttctcttcgaagttttcgacgtggtcagagtgcatcagccacaccgcggcatcatcgaggcagtctacctgcgtacaccgttctcggccggtaacgctaccacgtaagaagcttcttgcttcttgcaaatagcagctgcaaccatggcctgcggatcccaaaacggctccagcgagcaagagctcagagccattgtccaagacctgggttgcggaccctattttttgggaacctacgataagcgcttcccggggttcatggcccccgataagctcgcctgtgccattgtaaatacggccggacgtgagacggggggagagcactggttggctttcggttggaacccacgttctaacacctgctacctttttgatccttttggattctcggatgatcgtctcaaacagatttaccagtttgaatatgagggtctcctgcgccgcagcgctcttgctaccaaggaccgctgtattacgctggaaaaatctacccagaccgtgcagggtccccgttctgccgcctgcggacttttctgctgcatgttccttcacgcctttgtgcactggcctgaccgtcccatggacggaaaccccaccatgaaattgctaactggagtgccaaacaacatgcttcattctcctaaagtccagcccaccctgtgtgacaatcaaaaagcactctaccattttcttaatacccattcgccttattttcgctcccatcgtacacacatcgaaagggccactgcgttcgaccgtatggatgttcaataatgactcatgtaaacaacgtgttcaataaacatcactttatttttttacatgtatcaaggctctgcattacttatttatttacaagtcgaatgggttctgacgagaatcagaatgacccgcaggcagtgatacgttgcggaactgatacttgggttgccacttgaattcgggaatcaccaacttgggaaccggtatatcgggcaggatgtcactccacagctttctggtcagctgcaaagctccaagcaggtcaggagccgaaatcttgaaatcacaattaggaccagtgctttgagcgcgagagttgcggtacaccggattgcagcactgaaacaccatcagcgacggatgtctcacgcttgccagcacggtgggatctgcaatcatgcccacatccagatcttcagcattggcaatgctgaacggggtcatcttgcaggtctgcctacccatggcgggcacccaattaggcttgtggttgcaatcgcagtgcagggggatcagtatcatcttggcctgatcctgtctgattcctggatacacggctctcatgaaagcatcatattgcttgaaagcctgctgggctttactaccctcggtataaaacatcccgcaggacctgctcgaaaactggttagctgcacagccggcatcattcacacagcagcgggcgtcattgttagctatttgcaccacacttctgccccagcggttttgggtgattttggttcgctcgggattctcctttaaggctcgttgtccgttctcgctggccacatccatctcgataatctgctccttctgaatcataatattgccatgcaggcacttcagcttgccctcataatcattgcagccatgaggccacaacgcacagcctgtacattcccaattatggtgggcgatctgagaaaaagaatgtatcattccctgcagaaatcttcccatcatcgtgctcagtgtcttgtgactagtgaaagttaactggatgcctcggtgctcctcgtttacgtactggtgacagatgcgcttgtattgttcgtgttgctcaggcattagtttaaaagaggttctaagttcgttatccagcctgtacttctccatcagcagacacatcacttccatgcctttctcccaagcagacaccaggggcaagctaatcggattcttaacagtgcaggcagcagctcctttagccagagggtcatctttagcgatcttctcaatgcttcttttgccatccttctcaacgatgcgcacgggcgggtagctgaaacccactgctacaagttgcgcctcttctctttcttcttcgctgtcttgactgatgtcttgcatggggatatgtttggtcttccttggcttctttttggggggtatcggaggaggaggactgtcgctccgttccggagacagggaggattgtgacgtttcgctcaccattaccaactgactgtcggtagaagaacctgaccccacacggcgacaggtgtttctcttcgggggcagaggtggaggcgattgcgaagggctgcggtccgacctggaaggcggatgactggcagaaccccttccgcgttcgggggtgtgctccctgtggcggtcgcttaactgatttccttcgcggctggccattgtgttctcctaggcagagaaacaacagacatggaaactcagccattgctgtcaacatcgccacgagtgccatcacatctcgtcctcagcgacgaggaaaaggagcagagcttaagcattccaccgcccagtcctgccaccacctctaccctagaagataaggaggtcgacgcatctcatgacatgcagaataaaaaagcgaaagagtctgagacagacatcgagcaagacccgggctatgtgacaccggtggaacacgaggaagagttgaaacgctttctagagagagaggatgaaaactgcccaaaacaacgagcagataactatcaccaagatgctggaaatagggatcagaacaccgactacctcatagggcttgacggggaagacgcgctccttaaacatctagcaagacagtcgctcatagtcaaggatgcattattggacagaactgaagtgcccatcagtgtggaagagctcagccgcgcctacgagcttaacctcttttcacctcgtactccccccaaacgtcagccaaacggcacctgcgagccaaatcctcgcttaaacttttatccagcttttgctgtgccagaagtactggctacctatcacatcttttttaaaaatcaaaaaattccagtctcctgccgcgctaatcgcacccgcgccgatgccctactcaatctgggacctggttcacgcttacctgatatagcttccttggaagaggttccaaagatcttcgagggtctgggcaataatgagactcgggccgcaaatgctctgcaaaagggagaaaatggcatggatgagcatcacagcgttctggtggaattggaaggcgataatgccagactcgcagtactcaagcgaagcatcgaggtcacacacttcgcatatcccgctgtcaacctgccccctaaagtcatgacggcggtcatggaccagttactcattaagcgcgcaagtcccctttcagaagacatgcatgacccagatgcctgtgatgagggtaaaccagtggtcagtgatgagcagctaacccgatggctgggcaccgactctcccagggatttggaagagcgtcgcaagcttatgatggccgtggtgctggttaccgtagaactagagtgtctccgacgtttctttaccgattcagaaaccttgcgcaaactcgaagagaatctgcactacacttttagacacggctttgtgcggcaggcatgcaagatatctaacgtggaactcaccaacctggtttcctacatgggtattctgcatgagaatcgcctaggacaaagcgtgctgcacagcaccctgaagggggaagcccgccgtgattacatccgcgattgtgtctatctgtacctgtgccacacgtggcaaaccggcatgggtgtatggcagcaatgtttagaagaacagaacttgaaagagcttgacaagctcttacagaaatctcttaaggttctgtggacagggttcgacgagcgcaccgtcgcttccgacctggcagacctcatcttcccagagcgtctcagggttactttgcgaaacggattgcctgactttatgagccagagcatgcttaacaattttcgctctttcatcctggaacgctccggtatcctgcccgccacctgctgcgcactgccctccgactttgtgcctctcacctaccgcgagtgccccccgccgctatggagtcactgctacctgttccgtctggccaactatctctcctaccactcggatgtgatcgaggatgtgagcggagacggcttgctggagtgtcactgccgctgcaatctgtgcacgccccaccggtccctagcttgcaacccccagttgatgagcgaaacccagataataggcacctttgaattgcaaggccccagcagccaaggcgatgggtcttctcctgggcaaagtttaaaactgaccccgggactgtggacctccgcctacttgcgcaagtttgctccggaagattaccacccctatgaaatcaagttctatgaggaccaatcacagcctccaaaggccgaactttcggcctgcgtcatcacccagggggcaattctggcccaattgcaagccatccaaaaatcccgccaagaatttctactgaaaaagggtaagggggtctaccttgacccccagaccggcgaggaactcaacacaaggttccctcaggatgtcccaacgacgagaaaacaagaagttgaaggtgcagccgccgcccccagaagatatggaggaagattgggacagtcaggcagaggaggcggaggaggacagtctggaggacagtctggaggaagacagtttggaggaggaaaacgaggaggcagaggaggtggaagaagtaaccgccgacaaacagttatcctcggctgcggagacaagcaacagcgctaccatctccgctccgagtcgaggaacccggcggcgtcccagcagtagatgggacgagaccggacgcttcccgaacccaaccagcgcttccaagaccggtaagaaggatcggcagggatacaagtcctggcgggggcataagaatgccatcatctcctgcttgcatgagtgcgggggcaacatatccttcacgcggcgctacttgctattccaccatggggtgaactttccgcgcaatgttttgcattactaccgtcacctccacagcccctactatagccagcaaatcccggcagtctcgacagataaagacagcggcggcgacctccaacagaaaaccagcagcggcagttagaaaatacacaacaagtgcagcaacaggaggattaaagattacagccaacgagccagcgcaaacccgagagttaagaaatcggatctttccaaccctgtatgccatcttccagcagagtcggggtcaagagcaggaactgaaaataaaaaaccgatctctgcgttcgctcaccagaagttgtttgtatcacaagagcgaagatcaacttcagcgcactctcgaggacgccgaggctctcttcaacaagtactgcgcgctgactcttaaagagtaggcagcgaccgcgcttattcaaaaaaggcgggaattacatcatcctcgacatgagtaaagaaattcccacgccttacatgtggagttatcaaccccaaatgggattggcggcaggcgcctcccaggactactccacccgcatgaattggctcagcgccgggccttctatgatttctcgagttaatgatatacgcgcctaccgaaaccaaatacttttggaacagtcagctcttaccaccacgccccgccaacaccttaatcccagaaattggcccgccgccctagtgtaccaggaaagtcccgctcccaccactgtattacttcctcgagacgcccaggccgaagtccaaatgactaatgcaggtgcgcagttagctggcggctccaccctatgtcgtcacaggcctcggcataatataaaacgcctgatgatcagaggccgaggtatccagctcaacgacgagtcggtgagctctccgcttggtctacgaccagacggaatctttcagattgccggctgcgggagatcttccttcacccctcgtcaggctgttctgactttggaaagttcgtcttcgcaaccccgctcgggcggaatcgggaccgttcaatttgtggaggagtttactccctctgtctacttcaaccccttctccggatctcctgggcattacccggacgagttcataccgaacttcgacgcgattagcgagtcagtggacggctacgattgatgtctggtgacgcggctgagctatctcggctgcgacatctagaccactgccgccgctttcgctgctttgcccgggaactcattgagttcatctacttcgaactccccaaggatcaccctcaaggtccggcccacggagtgcggatttctatcgaaggcaaaatagactctcgcctgcaacgaattttctcccagcggcccgtgctgatcgagcgagaccagggaaacaccacggtttccatctactgcatttgtaatcaccccggattgcatgaaagcctttgctgtcttatgtgtactgagtttaataaaaactgaattaagactctcctacggactgccgcttcttcaacccggattttacaaccagaagaacgaaacttttcctgtcgtccaggactctgttaacttcacctttcctactcacaaactagaagctcaacgactacaccgcttttccagaagcattttccctactaatactactttcaaaaccggaggtgagctccaaggtcttcctacagaaaacccttgggtggaagcgggccttgtagtgctaggaattcttgcgggtgggcttgtgattattctttgctacctatacacaccttgcttcactttcttagtggtgttgtggtattggtttaaaaaatggggcccatactagtcttgcttgttttactttcgcttttggaaccgggttctgccaattacgatccatgtctagacttcgacccagaaaactgcacacttacttttgcacccgacacaagccgcatctgtggagttcatcgcctctcttacgaacttggcccccaacgacaaaaatttacctgcatggtgggaatcaaccccatagttatcacccagcaaagtggagatactaagggttgcattcactgctcctgcgattccatcgagtgcacctacaccctgctgaagaccctatgcggcctaagagacctgctaccaatgaattaaaaaatgattaataaaaaatcacttacttgaaatcagcaataaggtctctgttgaaattttctcccagcagcacctcacttccctcttcccaactctggtattctaaaccccgttcagcggcatactttctccatactttaaaggggatgtcaaattttagctcctctcctgtacccacaatcttcatgtctttcttcccagatgaccaagagagtccggctcagtgactccttcaaccctgtctacccctatgaagatgaaagcacctcccaacacccctttataaacccagggtttatttccccaaatggcttcacacaaagcccaaacggagttcttactttaaaatgtttaaccccactaacaaccacaggcggatctctacagctaaaagtgggagggggacttacagtggatgacaccaacggttttttgaaagaaaacataagtgccaccacaccactcgttaagactggtcactctataggtttaccactaggagccggattgggaacgaatgaaaataaactttgtatcaaattaggacaaggacttacattcaattcaaacaacatttgcattgatgacaatattaacaccttatggacaggagtcaaccccaccgaagccaactgtcaaatcatgaactccagtgaatctaatgattgcaaattaattctaacactagttaaaactggagcactagtcactgcatttgtttatgttataggagtatctaacaattttaatatgctaactacacacagaaatataaattttactgcagagctgtttttcgattctactggtaatttactaactagactctcatccctcaaaactccacttaatcataaatcaggacaaaacatggctactggtgccattactaatgctaaaggtttcatgcccagcacgactgcctatcctttcaatgataattctagagaaaaagaaaactacatttacggaacttgttactacacagctagtgatcgcactgcttttcccattgacatatctgtcatgcttaaccgaagagcaataaatgacgagacatcatattgtattcgtataacttggtcctggaacacaggagatgccccagaggtgcaaacctctgctacaaccctagtcacctccccatttaccttttactacatcagagaagacgactgacaaataaagtttgcgatcgccaggcccaccatggactggacctggaggatcctcttcttggtggcagcagccacaggagcccactcccaggtgcagctggtgcagtctggggctgaggtgaagaagcctggggcctcagtgaaggtctcctgcaaggcttctggatacaccttcaccggctactatatgcactgggtgcgacaggcccctggacaagggcttgagtggatgggatggatcaaccctgacagtggtggcacaaactatgcacagaagtttcagggcagggtcaccatgaccagggacacgtccatcagcacagcctacatggagctgaacaggctgagatctgacgacacggccgtgtattactgtgcgagagatcagcccctaggatattgtactaatggtgtatgctcctactttgactactggggccagggaaccctggtcaccgtctcctcagcctccaccaagggcccatcggtcttccccctggcgccctgctccaggagcacctccgagagcacagcggccctgggctgcctggtcaaggactacttccccgaaccggtgacggtgtcgtggaactcaggcgctctgaccagcggcgtgcacaccttcccagctgtcctacagtcctcaggactctactccctcagcagcgtggtgaccgtgccctccagcaacttcggcacccagacctacacctgcaacgtagatcacaagcccagcaacaccaaggtggacaagacagttgagcgcaaatgttgtgtcgagtgcccaccgtgcccagcaccacctgtggcaggaccgtcagtcttcctcttccccccaaaacccaaggacaccctcatgatctcccggacccctgaggtcacgtgcgtggtggtggacgtgagccacgaagaccccgaggtccagttcaactggtacgtggacggcgtggaggtgcataatgccaagacaaagccacgggaggagcagttcaacagcacgttccgtgtggtcagcgtcctcaccgttgtgcaccaggactggctgaacggcaaggagtacaagtgcaaggtctccaacaaaggcctcccagcccccatcgagaaaaccatctccaaaaccaaagggcagccccgagaaccacaggtgtacaccctgcccccatcccgggaggagatgaccaagaaccaggtcagcctgacctgcctggtcaaaggcttctaccccagcgacatcgccgtggagtgggagagcaatgggcagccggagaacaactacaagaccacacctcccatgctggactccgacggctccttcttcctctacagcaagctcaccgtggacaagagcaggtggcagcaggggaacgtcttctcatgctccgtgatgcatgaggctctgcacaaccactacacgcagaagagcctctccctgtctccgggtaaaggaagcggagctactaacttcagcctgctgaagcaggctggagacgtggaggagaaccctggacctaggctccctgctcagctcctggggctcctgctgctctggttcccaggttccagatgcgacatccagatgacccagtctccatcttccgtgtctgcatctgtaggagacagagtcaccatcacttgtcgggcgagtcagggtatttacagctggttagcctggtatcagcagaaaccagggaaagcccctaacctcctgatctatactgcatccactttacaaagtggggtcccatcaaggttcagcggcagtggatctgggacagatttcactctcaccatcagcagcctgcaacctgaagattttgcaacttactattgtcaacaggctaacattttcccgctcactttcggcggagggaccaaggtggagatcaaacgaactgtggctgcaccatctgtcttcatcttcccgccatctgatgagcagttgaaatctggaactgcctctgttgtgtgcctgctgaataacttctatcccagagaggccaaagtacagtggaaggtggataacgccctccaatcgggtaactcccaggagagtgtcacagagcaggacagcaaggacagcacctacagcctcagcagcaccctgacgctgagcaaagcagactacgagaaacacaaagtctacgcctgcgaagtcacccatcagggcctgagctcgcccgtcacaaagagcttcaacaggggagagtgttaggctagcttgactgactgagatacagcgtaccttcagctcacagacatgataagatacattgatgagtttggacaaaccacaactagaatgcagtgaaaaaaatgctttatttgtgaaatttgtgatgctattgctttatttgtaaccattataagctgcaataaacaagttaacaacaacaattgcattcattttatgtttcaggttcagggggaggtgtgggaggttttttaaagcaagtaaaacctctacaaatgtggtcctgcaggaacttgtttatttgaaaatcaattcacaaaatccgagtagttattttgcctcccccttcccatttaacagaatacaccaatctctccccacgcacagctttaaacatttggataccattagatatagacatggttttagattccacattccaaacagtttcagagcgagccaatctggggtcagtgatagataaaaatccatcgggatagtcttttaaagcgctttcacagtccaactgctgcggatgcgactccggagtctggatcacggtcatctggaagaagaacgatgggaatcataatccgaaaacggtatcggacgattgtgtctcatcaaacccacaagcagccgctgtctgcgtcgctccgtgcgactgctgtttatgggatcagggtccacagtgtcctgaagcatgattttaatagcccttaacatcaactttctggtgcgatgcgcgcagcaacgcattctgatttcactcaaatctttgcagtaggtacaacacattattacaatattgtttaataaaccataattaaaagcgctccagccaaaactcatatctgatataatcgcccctgcatgaccatcataccaaagtttaatataaattaaatgacgttccctcaaaaacacactacccacatacatgatctcttttggcatgtgcatattaacaatctgtctgtaccatggacaacgttggttaatcatgcaacccaatataaccttccggaaccacactgccaacaccgctcccccagccatgcattgaagtgaaccctgctgattacaatgacaatgaagaacccaattctctcgaccgtgaatcacttgagaatgaaaaatatctatagtggcacaacatagacataaatgcatgcatcttctcataatttttaactcctcaggatttagaaacatatcccagggaataggaagctcttgcagaacagtaaagctggcagaacaaggaagaccacgaacacaacttacactatgcatagtcatagtatcacaatctggcaacagcgggtggtcttcagtcatagaagctcgggtttcattttcctcacaacgtggtaactgggctctggtgtaagggtgatgtctggcgcatgatgtcgagcgtgcgcgcaaccttgtcataatggagttgcttcctgacattctcgtattttgtatagcaaaacgcggccctggcagaacacactcttcttcgccttctatcctgccgcttagcgtgttccgtgtgatagttcaagtacaaccacactcttaagttggtcaaaagaatgctggcttcagttgtaatcaaaactccatcgcatctaatcgttctgaggaaatcatccaagcaatgcaactggattgtgtttcaagcaggagaggagagggaagagacggaagaaccatgttaatttttattccaaacgatctcgcagtacttcaaattgtagatcgcgcagatggcatctctcgcccccactgtgttggtgaaaaagcacagctagatcaaaagaaatgcgattttcaaggtgctcaacggtggcttccagcaaagcctccacgcgcacatccaagaacaaaagaataccaaaagaaggagcattttctaactcctcaatcatcatattacattcctgcaccattcccagataattttcagctttccagccttgaattattcgtgtcagttcttgtggtaaatccaatccacacattacaaacaggtcccggagggcgccctccaccaccattcttaaacacaccctcataatgacaaaatatcttgctcctgtgtcacctgtagcgaattgagaatggcaacatcaattgacatgcccttggctctaagttcttctttaagttctagttgtaaaaactctctcatattatcaccaaactgcttagccagaagccccccgggaacaagagcaggggacgctacagtgcagtacaagcgcagacctccccaattggctccagcaaaaacaagattggaataagcatattgggaaccgccagtaatatcatcgaagttgctggaaatataatcaggcagagtttcttgtaaaaattgaataaaagaaaaatttgccaaaaaaacattcaaaacctctgggatgcaaatgcaataggttaccgcgctgcgctccaacattgttagttttgaattagtctgcaaaaataaaaaaaaaaacaagcgtcatatcatagtagcctgacgaacagatggataaatcagtctttccatcacaagacaagccacagggtctccagctcgaccctcgtaaaacctgtcatcatgattaaacaacagcaccgaaagttcctcgcggtgaccagcatgaataattcttgatgaagcatacaatccagacatgttagcatcagttaacgagaaaaaacagccaacatagcctttgggtataattatgcttaatcgtaagtatagcaaagccacccctcgcggatacaaagtaaaaggcacaggagaataaaaaatataattatttctctgctgctgttcaggcaacgtcgcccccggtccctctaaatacacatacaaagcctcatcagccatggcttaccagacaaagtacagcgggcacacaaagcacaagctctaaagtgactctccaacctctccacaatatatatatacacaagccctaaactgacgtaatgggagtaaagtgtaaaaaatcccgccaaacccaacacacaccccgaaactgcgtcaccagggaaaagtacagtttcacttccgcaatcccaacaggcgtaacttcctctttctcacggtacgtgatatcccactaacttgcaacgtcattttcccacggtcgcaccgccccttttagccgttaaccccacagccaatcaccacacgatccacactttttaaaatcacctcatttacatattggcaccattccatctataaggtatattatatagataga

SEQ ID NO: 14 - RNA, 13 nt, Artificial Sequence
  Kozak sequence
  misc_feature (7)..(7): R is purine, adenine or guanine
gccgccrccaugg

SEQ ID NO: 15 - DNA, 26 bp, Artificial Sequence
  splice acceptor sequence
tgctaatcttcctttctctcttcagg

SEQ ID NO: 16 - DNA, 14 bp, Artificial Sequence
  splice acceptor sequence
tttctctcttcagg

SEQ ID NO: 17 - DNA, 22 bp, Artificial Sequence
  Forward Primer
acggaacttgttactacacagc

SEQ ID NO: 18 - DNA, 21 bp, Artificial Sequence
  Reverse Primer
ctttcacagtccaactgctgc

SEQ ID NO: 19 - DNA, 22 bp, Artificial Sequence
  Forward Primer
agccggagaacaactacaagac

SEQ ID NO: 20 - DNA, 21 bp, Artificial Sequence
  Forward Primer
catccagatgacccagtctcc

SEQ ID NO: 21 - DNA, 24 bp, Artificial Sequence
  Reverse Primer
ggacaaaccacaactagaatgcag

SEQ ID NO: 22 - DNA, 20 bp, Artificial Sequence
  Forward primer
cctcagtgaaggtctcctgc

SEQ ID NO: 23 - DNA, 24 bp, Artificial Sequence
  Reverse Primer
ggacaaaccacaactagaatgcag

SEQ ID NO: 24 - protein, 22 aa, Artificial Sequence
  High efficiency self-cleavable P2A peptide sequence
GSGATNFSLLKQAGDVEENPGP

SEQ ID NO: 25 - protein, 21 aa, Artificial Sequence
  High efficiency self-cleavable F2A peptide sequence
GSGEGRGSLLTCGDVEENPGP

SEQ ID NO: 26 - protein, 23 aa, Artificial Sequence
  High efficiency self-cleavable E2A peptide sequence
GSGQCTNYALLKLAGDVESNPGP

SEQ ID NO: 27 - protein, 25 aa, Artificial Sequence
  High efficiency self-cleavable T2A peptide sequence
GSGVKQTLNFDLLKLAGDVESNPGP